European Patent Application EP 4 166 650 A1, published April 19, 2023. Title: MICROORGANISMS AND METHODS FOR PRODUCING SIALYLATED AND N-ACETYLGLUCOSAMINE-CONTAINING OLIGOSACCHARIDES. Applicant: Glycosyn LLC. The sequence listing filed with the application follows.

SEQUENCE LISTING (43 sequences)

SEQ ID NO: 1 - DNA, 5877 bp, Escherichia coli
  source 1..5877: mol_type = genomic DNA
gcagcggaactcacaaggcaccataacgtcccctccctgataacgctgatactgtggtcgcggttatgccagttggcatcttcacgtaaatagagcaaatagtcccgcgcctggctggcggtttgccatagccgttgcgactgctgccagtattgccagccatagagtccacttgcgcttagcatgaccaaaatcagcatcgcgaccagcgtttcaatcagcgtataaccacgttgtgttttcatgccggcagtatggagcgaggagaaaaaaagacgagggccagtttctatttcttcggcgcatcttccggactatttacgccgttgcaggacgttgcaaaatttcgggaaggcgtctcgaagaatttaacggagggtaaaaaaaccgacgcacactggcgtcggctctggcaggatgtttcgtaattagatagccaccggcgctttattaaacctactatgaccatgattacggattcactggccgtcgttttacaacgtcgtgactgggaaaaccctggcgttacccaacttaatcgccttgcagcacatccccctttcgccagctggcgtaatagcgaagaggcccgcaccgatcgcccttcccaacagttgcgcagcctgaatggcgaatggcgctttgcctggtttccggcaccagaagcggtgccggaaagctggctggagtgcgatcttcctgaggccgatactgtcgtcgtcccctcaaactggcagatgcacggttacgatgcgcccatctacaccaacgtgacctatcccattacggtcaatccgccgtttgttcccacggagaatccgacgggttgttactcgctcacatttaatgttgatgaaagctggctacaggaaggccagacgcgaattatttttgatggcgttaactcggcgtttcatctgtggtgcaacgggcgctgggtcggttacggccaggacagtcgtttgccgtctgaatttgacctgagcgcatttttacgcgccggagaaaaccgcctcgcggtgatggtgctgcgctggagtgacggcagttatctggaagatcaggatatgtggcggatgagcggcattttccgtgacgtctcgttgctgcataaaccgactacacaaatcagcgatttccatgttgccactcgctttaatgatgatttcagccgcgctgtactggaggctgaagttcagatgtgcggcgagttgcgtgactacctacgggtaacagtttctttatggcagggtgaaacgcaggtcgccagcggcaccgcgcctttcggcggtgaaattatcgatgagcgtggtggttatgccgatcgcgtcacactacgtctgaacgtcgaaaacccgaaactgtggagcgccgaaatcccgaatctctatcgtgcggtggttgaactgcacaccgccgacggcacgctgattgaagcagaagcctgcgatgtcggtttccgcgaggtgcggattgaaaatggtctgctgctgctgaacggcaagccgttgctgattcgaggcgttaaccgtcacgagcatcatcctctgcatggtcaggtcatggatgagcagacgatggtgcaggatatcctgctgatgaagcagaacaactttaacgccgtgcgctgttcgcattatccgaaccatccgctgtggtacacgctgtgcgaccgctacggcctgtatgtggtggatgaagccaatattgaaacccacggcatggtgccaatgaatcgtctgaccgatgatccgcgctggctaccggcgatgagcgaacgcgtaacgcgaatggtgcagcgcgatcgtaatcacccgagtgtgatcatctggtcgctggggaatgaatcaggccacggcgctaatcacgacgcgctgtatcgctggatcaaatctgtcgatccttcccgcccggtgcagtatgaaggcggcggagccgacaccacggccaccgatattatttgcccgatgtacgcgcgcgtggatgaagaccagcccttcccggctgtgccgaaatggtccatcaaaaaatggctttcgctacctggagagacgcgcccgctgatcctttgcgaatacgcccacgcgatgggtaacagtcttggcggtttcgctaaatactggcaggcgtttcgtcagtatccccgtttacagggcggcttcgtctgggactgggtggatcagtcgctgattaaatatgatgaaaacggcaacccgtggtcggcttacggcggtgattttggcgatacgccgaacgatcgccagttctgtatgaacggtctggtctttgccgaccgcacgccgcatccagcgctgacggaagcaaaacaccagcagcagtttttccagttccgtttatccgggcaaaccatcgaagtgaccagcgaatacctgttccgtcatagcgataacgagctcctgcactggatggtggcgctggatggtaagccgctggcaagcggtgaagtgcctctggatgtcgctccacaaggtaaacagttgattgaactgcctgaactaccgcagccggagagcgccgggcaactctggctcacagtacgcgtagtgcaaccgaacgcgaccgcatggtcagaagccgggcacatcagcgcctggcagcagtggcgtctggcggaaaacctcagtgtgacgctccccgccgcgtcccacgccatcccgcatctgaccaccagcgaaatggatttttgcatcgagctgggtaataagcgttggcaatttaaccgccagtcaggctttctttcacagatgtggattggcgataaaaaacaactgttgacgccgctgcgcgatcagttcacccgtgcaccgctggataacgacattggcgtaagtgaagcgacccgcattgaccctaacgcctgggtcgaacgctggaaggcggcgggccattaccaggccgaagcagcgttgttgcagtgcacggcagatacacttgctgatgcggtgctgattacgaccgctcacgcgtggcagcatcaggggaaaaccttatttatcagccggaaaacctaccggattgatggtagtggtcaaatggcgattaccgttgatgttgaagtggcgagcgatacaccgcatccggcgcggattggcctgaactgccagctggcgcaggtagcagagcgggtaaactggctcggattagggccgcaagaaaactatcccgaccgccttactgccgcctgttttgaccgctgggatctgccattgtcagacatgtataccccgtacgtcttcccgagcgaaaacggtctgcgctgcgggacgcgcgaattgaattatggcccacaccagtggcgcggcgacttccagttcaacatcagccgctacagtcaacagcaactgatggaaaccagccatcgccatctgctgcacgcggaagaaggcacatggctgaatatcgacggtttccatatggggattggtggcgacgactcctggagcccgtcagtatcggcggaattccagctgagcgccggtcgctaccattaccagttggtctggtgtcaaaaataagcggccgctttatgtaggctggagctgcttcgaagttcctatactttctagagaataggaacttcggaataggaacttcaagatccccttattagaagaactcgtcaagaaggcgatagaaggcgatgcgctgcgaatcgggagcggcgataccgtaaagcacgaggaagcggtcagcccattcgccgccaagctcttcagcaatatcacgggtagccaacgctatgtcctgatagcggtccgccacacccagccggccacagtcgatgaatcctgaaaagcggccattttccaccatgatattcggcaagcaggcatcgccatgggtcacgacgagatcctcgccgtcgggcatgcgcgccttgagcctggcgaacagttcggctggcgcgagcccctgatgctcttcgtccagatcatcctgatcgacaagaccggcttccatccgagtacgtgctcgctcgatgcgatgtttcgcttggtggtcgaatgggcaggtagccggatcaagcgtatgcagccgccgcattgcatcagccatgatggatactttctcggcaggagcaaggtgagatgacaggagatcctgccccggcacttcgcccaatagcagccagtcccttcccgcttcagtgacaacgtcgagcacagctgcgcaaggaacgcccgtcgtggccagccacgatagccgcgctgcctcgtcctgcagttcattcagggcaccggacaggtcggtcttgacaaaaagaaccgggcgcccctgcgctgacagccggaacacggcggcatcagagcagccgattgtctgttgtgcccagtcatagccgaatagcctctccacccaagcggccggagaacctgcgtgcaatccatcttgttcaatcatgcgaaacgatcctcatcctgtctcttgatcagatcttgatcccctgcgccatcagatccttggcggcaagaaagccatccagtttactttgcagggcttcccaaccttaccagagggcgccccagctggcaattccggttcgcttgctgtccataaaaccgcccagtctagctatcgccatgtaagcccactgcaagctacctgctttctctttgcgcttgcgttttcccttgtccagatagcccagtagctgacattcatccggggtcagcaccgtttctgcggactggctttctacgtgttccgcttcctttagcagcccttgcgccctgagtgcttgcggcagcgtgagcttcaaaagcgctctgaagttcctatactttctagagaataggaacttcgaactgcaggtcgacggatccccggaatcatggttcctcaggaaacgtgttgctgtgggctgcgacgatatgcccagaccatcatgatcacacccgcgacaatcatcgggatggaaagaatttgccccatgctgatgtactgcacccaggcaccggtaaactgcgcgtcgggctggcggaaaaactcaacaatgatgcgaaacgcgccgtaaccaatcaggaacaaacctgagacagctcccattgggcgtggtttacgaatatacaggttgaggataataaacagcaccacaccttccagcagcagctcgtaaagctgtgatgggtggcgcggcagcacaccgtaagtgtcgaaaatggattgccactgcgggttggtttgcagcagcaaaatatcttctgtacgggagccagggaacagcatggcaaacgggaagttcgggtcaacgcggccccacaattcaccgttaataaagttgcccagacgcccggcaccaagaccaaacggaatgagtggtgcgataaaatcagagacctggaagaaggaacgtttagtacggcgggcgaagataatcatcaccacgataacgccaatcaggccgccgtggaaagacatgccgccgtcccagacacggaacagatacagcggatcggccataaactgcgggaaattgtagaacagaacataaccaatacgtcccccgaggaagacgccgaggaagcccgcatagagtaagttttcaacttcatttttggtccagccgctgcccggacgattcgcccgtcgtgttgccagccacattgcaaaaatgaaacccaccagatacatcaggccgtaccagtgaagcgccacgggtcctattgagaaaatgaccggatcaaactccggaaaatgcagatagctactggtcatctgtcaccacaagttcttgttatttcgctgaaagagaacagcgattgaaatgcgcgccgcaggtttcaggcgctccaaaggtgcgaataatagcacaaggggacctggctggttgccggataccgttaaaagatatgtata

SEQ ID NO: 2 - DNA, 5409 bp, synthetic construct
  misc_feature 1..5409: note = engineered plasmid
  source 1..5409: mol_type = other DNA
tcgcgcgtttcggtgatgacggtgaaaacctctgacacatgcagctcccggagacggtcacagcttgtctgtaagcggatgccgggagcagacaagcccgtcagggcgcgtcagcgggtgttggcgggtgtcggggctggcttaactatgcggcatcagagcagattgtactgagagtgcaccatatatgcggtgtgaaataccgcacagatgcgtaaggagaaaataccgcatcaggcgcctcctcaacctgtatattcgtaaaccacgcccaatgggagctgtctcaggtttgttcctgattggttacggcgcgtttcgcatcattgttgagtttttccgccagcccgacgcgcagtttaccggtgcctgggtgcagtacatcagcatggggcaaattctttccatcccgatgattgtcgcgggtgtgatcatgatggtctgggcatatcgtcgcagcccacagcaacacgtttcctgaggaaccatgaaacagtatttagaactgatgcaaaaagtgctcgacgaaggcacacagaaaaacgaccgtaccggaaccggaacgctttccatttttggtcatcagatgcgttttaacctgcaagatggattcccgctggtgacaactaaacgttgccacctgcgttccatcatccatgaactgctgtggtttctgcagggcgacactaacattgcttatctacacgaaaacaatgtcaccatctgggacgaatgggccgatgaaaacggcgacctcgggccagtgtatggtaaacagtggcgcgcctggccaacgccagatggtcgtcatattgaccagatcactacggtactgaaccagctgaaaaacgacccggattcgcgccgcattattgtttcagcgtggaacgtaggcgaactggataaaatggcgctggcaccgtgccatgcattcttccagttctatgtggcagacggcaaactctcttgccagctttatcagcgctcctgtgacgtcttcctcggcctgccgttcaacattgccagctacgcgttattggtgcatatgatggcgcagcagtgcgatctggaagtgggtgattttgtctggaccggtggcgacacgcatctgtacagcaaccatatggatcaaactcatctgcaattaagccgcgaaccgcgtccgctgccgaagttgattatcaaacgtaaacccgaatccatcttcgactaccgtttcgaagactttgagattgaaggctacgatccgcatccgggcattaaagcgccggtggctatctaattacgaaacatcctgccagagccgacgccagtgtgcgtcggtttttttaccctccgttaaattcttcgagacgccttcccgaaggcgccattcgccattcaggctgcgcaactgttgggaagggcgatcggtgcgggcctcttcgctattacgccagctggcgaaagggggatgtgctgcaaggcgattaagttgggtaacgccagggttttcccagtcacgacgttgtaaaacgacggccagtgccaagcttactgctcacaagaaaaaaggcacgtcatctgacgtgccttttttatttgtactaccctgtacgattactgcaggtcgactctagatgcatgctcgagtcaacggtttttcagcaatcggtgcaaaatgccgaagtattgcctcaaggtaaacagccgccgcatcctgccgtctgccgcaaaatccagccacgcgccggcgggcagcgtgtccgtccgtttgaagcattggtacaaaaaccggcgggcgcgttcaaaatcttcttccggcaaatgtttctccagcaattcatacgctactgcttttatttggcggtattcaaggctgtcgaaccgggttttaaaacccatagactgcaaaaaatcgtttctggcggttttttggatgccttgcgcgatttcgtgttggcggatgctgtatttggatgaaacctgattggcgtgaaggcggtatttgaccaaggcttcgggataataagccagcctgcccaatttgctgacatcgtaccaaaattggtaatcttccgcccaatcccgctcggtgttgtaacgcaaaccgccgtcaatgacgctgcgcctcataatcatcgtgttgttgtgtatggggttgccgaaagggaaaaagtcggcaatgtcttcgtgtcgggtcggttttttccaaattttgccgtgttcgtggtgccgcgccagccggttgccgtccttttcttccgacaaaacttccagccacgcacccatcgcgatgatgctgcggtctttttccatctcacccacgattttctcaatccagtcgggggcggcaatatcgtctgcatcggtgcgcgcaatatattccccccccccccccgactttgccaattcatccagcccgatgtttaaagagggaatcagaccggaattgcgcggctgcgcgaggatgcggatgcggccgtcctgttcttggaaacgctgggcaatggcaagcgtaccgtccgtcgagccgtcatcgacaatcaaaatatccaagttgcgccaagtttgattcacgacggcggctaatgattgggcgaaatatttttctacgttgtaggcgcaaatcaatacgctgactaaaggctgcaatttattctcccgataggcacgatgccgtctgaaggcttcagacggcatatgtatatctccttcttgaattctaacaattgattgaatgtatgcaaataaatgcatacaccataggtgtggtttaatttgatgccctttttcagggctggaatgtgtaagagcggggttatttatgctgttgtttttttgttactcgggaagggctttacctcttccgcataaacgcttccatcagcgtttatagttaaaaaaatctttcggaactggttttgcgcttaccccaaccaacaggggatttgctgctttccattgagcctgtttctctgcgcgacgttcgcggcggcgtgtttgtgcatccatctggattctcctgtcagttagctttggtggtgtgtggcagttgtagtcctgaacgaaaaccccccgcgattggcacattggcagctaatccggaatcgcacttacggccaatgcttcgtttcgtatcacacaccccaaagccttctgctttgaatgctgcccttcttcagggcttaatttttaagagcgtcaccttcatggtggtcagtgcgtcctgctgatgtgctcagtatcaccgccagtggtatttatgtcaacaccgccagagataatttatcaccgcagatggttatctgtatgttttttatatgaatttattttttgcaggggggcattgtttggtaggtgagagatcaattctgcattaatgaatcggccaacgcgcggggagaggcggtttgcgtattgggcgctcttccgcttcctcgctcactgactcgctgcgctcggtcgttcggctgcggcgagcggtatcagctcactcaaaggcggtaatacggttatccacagaatcaggggataacgcaggaaagaacatgtgagcaaaaggccagcaaaaggccaggaaccgtaaaaaggccgcgttgctggcgtttttccataggctccgcccccctgacgagcatcacaaaaatcgacgctcaagtcagaggtggcgaaacccgacaggactataaagataccaggcgtttccccctggaagctccctcgtgcgctctcctgttccgaccctgccgcttaccggatacctgtccgcctttctcccttcgggaagcgtggcgctttctcatagctcacgctgtaggtatctcagttcggtgtaggtcgttcgctccaagctgggctgtgtgcacgaaccccccgttcagcccgaccgctgcgccttatccggtaactatcgtcttgagtccaacccggtaagacacgacttatcgccactggcagcagccactggtaacaggattagcagagcgaggtatgtaggcggtgctacagagttcttgaagtggtggcctaactacggctacactagaaggacagtatttggtatctgcgctctgctgaagccagttaccttcggaaaaagagttggtagctcttgatccggcaaacaaaccaccgctggtagcggtggtttttttgtttgcaagcagcagattacgcgcagaaaaaaaggatctcaagaagatcctttgatcttttctacggggtctgacgctcagtggaacgaaaactcacgttaagggattttggtcatgagattatcaaaaaggatcttcacctagatccttttaaattaaaaatgaagttttaaatcaatctaaagtatatatgagtaaacttggtctgacagttaccaatgcttaatcagtgaggcacctatctcagcgatctgtctatttcgttcatccatagttgcctgactccccgtcgtgtagataactacgatacgggagggcttaccatctggccccagtgctgcaatgataccgcgagacccacgctcaccggctccagatttatcagcaataaaccagccagccggaagggccgagcgcagaagtggtcctgcaactttatccgcctccatccagtctattaattgttgccgggaagctagagtaagtagttcgccagttaatagtttgcgcaacgttgttgccattgctacaggcatcgtggtgtcacgctcgtcgtttggtatggcttcattcagctccggttcccaacgatcaaggcgagttacatgatcccccatgttgtgcaaaaaagcggttagctccttcggtcctccgatcgttgtcagaagtaagttggccgcagtgttatcactcatggttatggcagcactgcataattctcttactgtcatgccatccgtaagatgcttttctgtgactggtgagtactcaaccaagtcattctgagaatagtgtatgcggcgaccgagttgctcttgcccggcgtcaatacgggataataccgcgccacatagcagaactttaaaagtgctcatcattggaaaacgttcttcggggcgaaaactctcaaggatcttaccgctgttgagatccagttcgatgtaacccactcgtgcacccaactgatcttcagcatcttttactttcaccagcgtttctgggtgagcaaaaacaggaaggcaaaatgccgcaaaaaagggaataagggcgacacggaaatgttgaatactcatactcttcctttttcaatattattgaagcatttatcagggttattgtctcatgagcggatacatatttgaatgtatttagaaaaataaacaaataggggttccgcgcacatttccccgaaaagtgccacctgacgtctaagaaaccattattatcatgacattaacctataaaaataggcgtatcacgaggccctttcgtc

SEQ ID NO: 3 - DNA, 6233 bp, synthetic construct
  misc_feature 1..6233: note = engineered plasmid
  source 1..6233: mol_type = other DNA
tcgcgcgtttcggtgatgacggtgaaaacctctgacacatgcagctcccggagacggtcacagcttgtctgtaagcggatgccgggagcagacaagcccgtcagggcgcgtcagcgggtgttggcgggtgtcggggctggcttaactatgcggcatcagagcagattgtactgagagtgcaccatatatgcggtgtgaaataccgcacagatgcgtaaggagaaaataccgcatcaggcgcctcctcaacctgtatattcgtaaaccacgcccaatgggagctgtctcaggtttgttcctgattggttacggcgcgtttcgcatcattgttgagtttttccgccagcccgacgcgcagtttaccggtgcctgggtgcagtacatcagcatggggcaaattctttccatcccgatgattgtcgcgggtgtgatcatgatggtctgggcatatcgtcgcagcccacagcaacacgtttcctgaggaaccatgaaacagtatttagaactgatgcaaaaagtgctcgacgaaggcacacagaaaaacgaccgtaccggaaccggaacgctttccatttttggtcatcagatgcgttttaacctgcaagatggattcccgctggtgacaactaaacgttgccacctgcgttccatcatccatgaactgctgtggtttctgcagggcgacactaacattgcttatctacacgaaaacaatgtcaccatctgggacgaatgggccgatgaaaacggcgacctcgggccagtgtatggtaaacagtggcgcgcctggccaacgccagatggtcgtcatattgaccagatcactacggtactgaaccagctgaaaaacgacccggattcgcgccgcattattgtttcagcgtggaacgtaggcgaactggataaaatggcgctggcaccgtgccatgcattcttccagttctatgtggcagacggcaaactctcttgccagctttatcagcgctcctgtgacgtcttcctcggcctgccgttcaacattgccagctacgcgttattggtgcatatgatggcgcagcagtgcgatctggaagtgggtgattttgtctggaccggtggcgacacgcatctgtacagcaaccatatggatcaaactcatctgcaattaagccgcgaaccgcgtccgctgccgaagttgattatcaaacgtaaacccgaatccatcttcgactaccgtttcgaagactttgagattgaaggctacgatccgcatccgggcattaaagcgccggtggctatctaattacgaaacatcctgccagagccgacgccagtgtgcgtcggtttttttaccctccgttaaattcttcgagacgccttcccgaaggcgccattcgccattcaggctgcgcaactgttgggaagggcgatcggtgcgggcctcttcgctattacgccagctggcgaaagggggatgtgctgcaaggcgattaagttgggtaacgccagggttttcccagtcacgacgttgtaaaacgacggccagtgccaagcttactgctcacaagaaaaaaggcacgtcatctgacgtgccttttttatttgtactaccctgtacgattactgcaggtcgactctagatgcatgctcgagttattatttaatatatttacaatagatgaaggacgcaatcgtacggataccgccgaacaggtagttaatgttaccggtcaggaagaagcacttcattttgataaccaggtcgttaaccatcaccatgtacaggtttttttttgcggtagactgaccttcgtgcaggcggtagtagaacaggtattccggcaggttttggaacttgatttttgccaggctcagacggttccacagctcgtaatcttcggagtagttagaaaacatataaccaccgatgctcgcgatgacttttttacgaaacattacgctcgggtgaacaatacaacacttatacggcaggtttttaacgatgtccaggttctcttccggcagtttggtcttgttgatttcacgacctttgtcgtcaataaagattgcgttggtacccacaacatctacgtacggattgttcttcaggaagtcaacctgtttagtaaaacggtccgggtgagagatgtcgtcagagtccatacgggcaataaattcgccgttgctcaggtcgatcgctttgttcagggagtacggcaggtaagcgatgttagtgcggatcagtttgattttgtcgttaactttgtgtttcagttcgttatagaagtcgtcagtgcagcagttcgcaacgatgatgatttcgaagctgctgaaggtctgagacaggatgctgttgatcgcttcgtccagaaaagggtttttcttgttaacaggcaggataacgctcacaaccgggtgggtagattccgcggattccgcttcatcgatgatcatatgtatatctccttcttctcgagtcaacggtttttcagcaatcggtgcaaaatgccgaagtattgcctcaaggtaaacagccgccgcatcctgccgtctgccgcaaaatccagccacgcgccggcgggcagcgtgtccgtccgtttgaagcattggtacaaaaaccggcgggcgcgttcaaaatcttcttccggcaaatgtttctccagcaattcatacgctactgcttttatttggcggtattcaaggctgtcgaaccgggttttaaaacccatagactgcaaaaaatcgtttctggcggttttttggatgccttgcgcgatttcgtgttggcggatgctgtatttggatgaaacctgattggcgtgaaggcggtatttgaccaaggcttcgggataataagccagcctgcccaatttgctgacatcgtaccaaaattggtaatcttccgcccaatcccgctcggtgttgtaacgcaaaccgccgtcaatgacgctgcgcctcataatcatcgtgttgttgtgtatggggttgccgaaagggaaaaagtcggcaatgtcttcgtgtcgggtcggttttttccaaattttgccgtgttcgtggtgccgcgccagccggttgccgtccttttcttccgacaaaacttccagccacgcacccatcgcgatgatgctgcggtctttttccatctcacccacgattttctcaatccagtcgggggcggcaatatcgtctgcatcggtgcgcgcaatatattccccccccccccccgactttgccaattcatccagcccgatgtttaaagagggaatcagaccggaattgcgcggctgcgcgaggatgcggatgcggccgtcctgttcttggaaacgctgggcaatggcaagcgtaccgtccgtcgagccgtcatcgacaatcaaaatatccaagttgcgccaagtttgattcacgacggcggctaatgattgggcgaaatatttttctacgttgtaggcgcaaatcaatacgctgactaaaggctgcaatttattctcccgataggcacgatgccgtctgaaggcttcagacggcatatgtatatctccttcttgaattctaacaattgattgaatgtatgcaaataaatgcatacaccataggtgtggtttaatttgatgccctttttcagggctggaatgtgtaagagcggggttatttatgctgttgtttttttgttactcgggaagggctttacctcttccgcataaacgcttccatcagcgtttatagttaaaaaaatctttcggaactggttttgcgcttaccccaaccaacaggggatttgctgctttccattgagcctgtttctctgcgcgacgttcgcggcggcgtgtttgtgcatccatctggattctcctgtcagttagctttggtggtgtgtggcagttgtagtcctgaacgaaaaccccccgcgattggcacattggcagctaatccggaatcgcacttacggccaatgcttcgtttcgtatcacacaccccaaagccttctgctttgaatgctgcccttcttcagggcttaatttttaagagcgtcaccttcatggtggtcagtgcgtcctgctgatgtgctcagtatcaccgccagtggtatttatgtcaacaccgccagagataatttatcaccgcagatggttatctgtatgttttttatatgaatttattttttgcaggggggcattgtttggtaggtgagagatcaattctgcattaatgaatcggccaacgcgcggggagaggcggtttgcgtattgggcgctcttccgcttcctcgctcactgactcgctgcgctcggtcgttcggctgcggcgagcggtatcagctcactcaaaggcggtaatacggttatccacagaatcaggggataacgcaggaaagaacatgtgagcaaaaggccagcaaaaggccaggaaccgtaaaaaggccgcgttgctggcgtttttccataggctccgcccccctgacgagcatcacaaaaatcgacgctcaagtcagaggtggcgaaacccgacaggactataaagataccaggcgtttccccctggaagctccctcgtgcgctctcctgttccgaccctgccgcttaccggatacctgtccgcctttctcccttcgggaagcgtggcgctttctcatagctcacgctgtaggtatctcagttcggtgtaggtcgttcgctccaagctgggctgtgtgcacgaaccccccgttcagcccgaccgctgcgccttatccggtaactatcgtcttgagtccaacccggtaagacacgacttatcgccactggcagcagccactggtaacaggattagcagagcgaggtatgtaggcggtgctacagagttcttgaagtggtggcctaactacggctacactagaaggacagtatttggtatctgcgctctgctgaagccagttaccttcggaaaaagagttggtagctcttgatccggcaaacaaaccaccgctggtagcggtggtttttttgtttgcaagcagcagattacgcgcagaaaaaaaggatctcaagaagatcctttgatcttttctacggggtctgacgctcagtggaacgaaaactcacgttaagggattttggtcatgagattatcaaaaaggatcttcacctagatccttttaaattaaaaatgaagttttaaatcaatctaaagtatatatgagtaaacttggtctgacagttaccaatgcttaatcagtgaggcacctatctcagcgatctgtctatttcgttcatccatagttgcctgactccccgtcgtgtagataactacgatacgggagggcttaccatctggccccagtgctgcaatgataccgcgagacccacgctcaccggctccagatttatcagcaataaaccagccagccggaagggccgagcgcagaagtggtcctgcaactttatccgcctccatccagtctattaattgttgccgggaagctagagtaagtagttcgccagttaatagtttgcgcaacgttgttgccattgctacaggcatcgtggtgtcacgctcgtcgtttggtatggcttcattcagctccggttcccaacgatcaaggcgagttacatgatcccccatgttgtgcaaaaaagcggttagctccttcggtcctccgatcgttgtcagaagtaagttggccgcagtgttatcactcatggttatggcagcactgcataattctcttactgtcatgccatccgtaagatgcttttctgtgactggtgagtactcaaccaagtcattctgagaatagtgtatgcggcgaccgagttgctcttgcccggcgtcaatacgggataataccgcgccacatagcagaactttaaaagtgctcatcattggaaaacgttcttcggggcgaaaactctcaaggatcttaccgctgttgagatccagttcgatgtaacccactcgtgcacccaactgatcttcagcatcttttactttcaccagcgtttctgggtgagcaaaaacaggaaggcaaaatgccgcaaaaaagggaataagggcgacacggaaatgttgaatactcatactcttcctttttcaatattattgaagcatttatcagggttattgtctcatgagcggatacatatttgaatgtatttagaaaaataaacaaataggggttccgcgcacatttccccgaaaagtgccacctgacgtctaagaaaccattattatcatgacattaacctataaaaataggcgtatcacgaggccctttcgtc

SEQ ID NO: 4 - DNA, 6254 bp, synthetic construct
  misc_feature 1..6254: note = engineered plasmid
  source 1..6254: mol_type = other DNA
tcgcgcgtttcggtgatgacggtgaaaacctctgacacatgcagctcccggagacggtcacagcttgtctgtaagcggatgccgggagcagacaagcccgtcagggcgcgtcagcgggtgttggcgggtgtcggggctggcttaactatgcggcatcagagcagattgtactgagagtgcaccatatatgcggtgtgaaataccgcacagatgcgtaaggagaaaataccgcatcaggcgcctcctcaacctgtatattcgtaaaccacgcccaatgggagctgtctcaggtttgttcctgattggttacggcgcgtttcgcatcattgttgagtttttccgccagcccgacgcgcagtttaccggtgcctgggtgcagtacatcagcatggggcaaattctttccatcccgatgattgtcgcgggtgtgatcatgatggtctgggcatatcgtcgcagcccacagcaacacgtttcctgaggaaccatgaaacagtatttagaactgatgcaaaaagtgctcgacgaaggcacacagaaaaacgaccgtaccggaaccggaacgctttccatttttggtcatcagatgcgttttaacctgcaagatggattcccgctggtgacaactaaacgttgccacctgcgttccatcatccatgaactgctgtggtttctgcagggcgacactaacattgcttatctacacgaaaacaatgtcaccatctgggacgaatgggccgatgaaaacggcgacctcgggccagtgtatggtaaacagtggcgcgcctggccaacgccagatggtcgtcatattgaccagatcactacggtactgaaccagctgaaaaacgacccggattcgcgccgcattattgtttcagcgtggaacgtaggcgaactggataaaatggcgctggcaccgtgccatgcattcttccagttctatgtggcagacggcaaactctcttgccagctttatcagcgctcctgtgacgtcttcctcggcctgccgttcaacattgccagctacgcgttattggtgcatatgatggcgcagcagtgcgatctggaagtgggtgattttgtctggaccggtggcgacacgcatctgtacagcaaccatatggatcaaactcatctgcaattaagccgcgaaccgcgtccgctgccgaagttgattatcaaacgtaaacccgaatccatcttcgactaccgtttcgaagactttgagattgaaggctacgatccgcatccgggcattaaagcgccggtggctatctaattacgaaacatcctgccagagccgacgccagtgtgcgtcggtttttttaccctccgttaaattcttcgagacgccttcccgaaggcgccattcgccattcaggctgcgcaactgttgggaagggcgatcggtgcgggcctcttcgctattacgccagctggcgaaagggggatgtgctgcaaggcgattaagttgggtaacgccagggttttcccagtcacgacgttgtaaaacgacggccagtgccaagcttactgctcacaagaaaaaaggcacgtcatctgacgtgccttttttatttgtactaccctgtacgattactgcaggtcgactctagatgcatgctcgagttatacaaactgccaatatttcaaatatttaaaatggagttctctcattaaggcgattttagggctataaggttcttcttttcgtgctatcgtagagatttgctcatcatcagcgatcacaaaaggttgtaacaccagatttttcacgccatggataaaagtagcgtccattatcgtatccacaggaacaacccattttcggctgcatttcaaaaaaactttggcaatcttaggcgtgatcacatagccttgagtccccaccccttcgctataagctttaatgatccccacacgctcttgtatctcgtggtttttatggctcaatggctcactttttacactggcatcatacaataaatgcatcaagcggatatagcctaactcttggatgtgtttttctaaaaaatccaagccctctttaaaatcctctttcaaggttatatcgtcttctaaaatacagatcgcttcattgagttctatgcatttttcccacaaggaataatgactcgcatagcacccaagctcccccaagctcataaacttcgcatggtattttaaagcgtaataaaacttagaaacctcactgatgagattggttgtaatccccatgtctttgatgttttgcgtgatgaaataagggtgtaaatgctttttcactaaggggtgcaacccgccttcaaaagttttagaataaatcgcatcaaaaatttgcgcttggtggtgggtggcattgatgctattgagtaaagttgtggtgtctctaaaaactaaaccaaatgtatcgcacactttttgatttaaagaaatggcaaaaacacgcatatgtatatctccttcttctcgagtcaacggtttttcagcaatcggtgcaaaatgccgaagtattgcctcaaggtaaacagccgccgcatcctgccgtctgccgcaaaatccagccacgcgccggcgggcagcgtgtccgtccgtttgaagcattggtacaaaaaccggcgggcgcgttcaaaatcttcttccggcaaatgtttctccagcaattcatacgctactgcttttatttggcggtattcaaggctgtcgaaccgggttttaaaacccatagactgcaaaaaatcgtttctggcggttttttggatgccttgcgcgatttcgtgttggcggatgctgtatttggatgaaacctgattggcgtgaaggcggtatttgaccaaggcttcgggataataagccagcctgcccaatttgctgacatcgtaccaaaattggtaatcttccgcccaatcccgctcggtgttgtaacgcaaaccgccgtcaatgacgctgcgcctcataatcatcgtgttgttgtgtatggggttgccgaaagggaaaaagtcggcaatgtcttcgtgtcgggtcggttttttccaaattttgccgtgttcgtggtgccgcgccagccggttgccgtccttttcttccgacaaaacttccagccacgcacccatcgcgatgatgctgcggtctttttccatctcacccacgattttctcaatccagtcgggggcggcaatatcgtctgcatcggtgcgcgcaatatattccccccccccccccgactttgccaattcatccagcccgatgtttaaagagggaatcagaccggaattgcgcggctgcgcgaggatgcggatgcggccgtcctgttcttggaaacgctgggcaatggcaagcgtaccgtccgtcgagccgtcatcgacaatcaaaatatccaagttgcgccaagtttgattcacgacggcggctaatgattgggcgaaatatttttctacgttgtaggcgcaaatcaatacgctgactaaaggctgcaatttattctcccgataggcacgatgccgtctgaaggcttcagacggcatatgtatatctccttcttgaattctaacaattgattgaatgtatgcaaataaatgcatacaccataggtgtggtttaatttgatgccctttttcagggctggaatgtgtaagagcggggttatttatgctgttgtttttttgttactcgggaagggctttacctcttccgcataaacgcttccatcagcgtttatagttaaaaaaatctttcggaactggttttgcgcttaccccaaccaacaggggatttgctgctttccattgagcctgtttctctgcgcgacgttcgcggcggcgtgtttgtgcatccatctggattctcctgtcagttagctttggtggtgtgtggcagttgtagtcctgaacgaaaaccccccgcgattggcacattggcagctaatccggaatcgcacttacggccaatgcttcgtttcgtatcacacaccccaaagccttctgctttgaatgctgcccttcttcagggcttaatttttaagagcgtcaccttcatggtggtcagtgcgtcctgctgatgtgctcagtatcaccgccagtggtatttatgtcaacaccgccagagataatttatcaccgcagatggttatctgtatgttttttatatgaatttattttttgcaggggggcattgtttggtaggtgagagatcaattctgcattaatgaatcggccaacgcgcggggagaggcggtttgcgtattgggcgctcttccgcttcctcgctcactgactcgctgcgctcggtcgttcggctgcggcgagcggtatcagctcactcaaaggcggtaatacggttatccacagaatcaggggataacgcaggaaagaacatgtgagcaaaaggccagcaaaaggccaggaaccgtaaaaaggccgcgttgctggcgtttttccataggctccgcccccctgacgagcatcacaaaaatcgacgctcaagtcagaggtggcgaaacccgacaggactataaagataccaggcgtttccccctggaagctccctcgtgcgctctcctgttccgaccctgccgcttaccggatacctgtccgcctttctcccttcgggaagcgtggcgctttctcatagctcacgctgtaggtatctcagttcggtgtaggtcgttcgctccaagctgggctgtgtgcacgaaccccccgttcagcccgaccgctgcgccttatccggtaactatcgtcttgagtccaacccggtaagacacgacttatcgccactggcagcagccactggtaacaggattagcagagcgaggtatgtaggcggtgctacagagttcttgaagtggtggcctaactacggctacactagaaggacagtatttggtatctgcgctctgctgaagccagttaccttcggaaaaagagttggtagctcttgatccggcaaacaaaccaccgctggtagcggtggtttttttgtttgcaagcagcagattacgcgcagaaaaaaaggatctcaagaagatcctttgatcttttctacggggtctgacgctcagtggaacgaaaactcacgttaagggattttggtcatgagattatcaaaaaggatcttcacctagatccttttaaattaaaaatgaagttttaaatcaatctaaagtatatatgagtaaacttggtctgacagttaccaatgcttaatcagtgaggcacctatctcagcgatctgtctatttcgttcatccatagttgcctgactccccgtcgtgtagataactacgatacgggagggcttaccatctggccccagtgctgcaatgataccgcgagacccacgctcaccggctccagatttatcagcaataaaccagccagccggaagggccgagcgcagaagtggtcctgcaactttatccgcctccatccagtctattaattgttgccgggaagctagagtaagtagttcgccagttaatagtttgcgcaacgttgttgccattgctacaggcatcgtggtgtcacgctcgtcgtttggtatggcttcattcagctccggttcccaacgatcaaggcgagttacatgatcccccatgttgtgcaaaaaagcggttagctccttcggtcctccgatcgttgtcagaagtaagttggccgcagtgttatcactcatggttatggcagcactgcataattctcttactgtcatgccatccgtaagatgcttttctgtgactggtgagtactcaaccaagtcattctgagaatagtgtatgcggcgaccgagttgctcttgcccggcgtcaatacgggataataccgcgccacatagcagaactttaaaagtgctcatcattggaaaacgttcttcggggcgaaaactctcaaggatcttaccgctgttgagatccagttcgatgtaacccactcgtgcacccaactgatcttcagcatcttttactttcaccagcgtttctgggtgagcaaaaacaggaaggcaaaatgccgcaaaaaagggaataagggcgacacggaaatgttgaatactcatactcttcctttttcaatattattgaagcatttatcagggttattgtctcatgagcggatacatatttgaatgtatttagaaaaataaacaaataggggttccgcgcacatttccccgaaaagtgccacctgacgtctaagaaaccattattatcatgacattaacctataaaaataggcgtatcacgaggccctttcgtc

SEQ ID NO: 5 - DNA, 7680 bp, synthetic construct
  misc_feature 1..7680: note = engineered plasmid
  source 1..7680: mol_type = other DNA
gtacccagcttttgttccctttagtgagggttaattgcgcgcttggcgtaatcatggtcatagctgtttcctgtgtgaaattgttatccgctcacaattccacacaacatacgagccggaagcataaagtgtaaagcctggggtgcctaatgagtgagctaactcacattaattgcgttgcgctcactgcccgctttccagtcgggaaacctgtcgtgccagctgcattaatgaatcggccaacgcgcggggagaggcggtttgcgtattgggcgcatgcataaaaactgttgtaattcattaagcattctgccgacatggaagccatcacaaacggcatgatgaacctgaatcgccagcggcatcagcaccttgtcgccttgcgtataatatttgcccatggtgaaaacgggggcgaagaagttgtccatattggccacgtttaaatcaaaactggtgaaactcacccagggattggctgagacgaaaaacatattctcaataaaccctttagggaaataggccaggttttcaccgtaacacgccacatcttgcgaatatatgtgtagaaactgccggaaatcgtcgtggtattcactccagagcgatgaaaacgtttcagtttgctcatggaaaacggtgtaacaagggtgaacactatcccatatcaccagctcaccgtctttcattgccatacggaattccggatgagcattcatcaggcgggcaagaatgtgaataaaggccggataaaacttgtgcttatttttctttacggtctttaaaaaggccgtaatatccagctgaacggtctggttataggtacattgagcaactgactgaaatgcctcaaaatgttctttacgatgccattgggatatatcaacggtggtatatccagtgatttttttctccattttagcttccttagctcctgaaaatctcgataactcaaaaaatacgcccggtagtgatcttatttcattatggtgaaagttggaacctcttacgtgccgatcaacgtctcattttcgccaaaagttggcccagggcttcccggtatcaacagggacaccaggatttatttattctgcgaagtgatcttccgtcacaggtatttattcgaagacgaaagggcctcgtgatacgcctatttttataggttaatgtcatgataataatggtttcttagacgtcaggtggcacttttcggggaaatgtgcgcgcccgcgttcctgctggcgctgggcctgtttctggcgctggacttcccgctgttccgtcagcagcttttcgcccacggccttgatgatcgcggcggccttggcctgcatatcccgattcaacggccccagggcgtccagaacgggcttcaggcgctcccgaaggtctcgggccgtctcttgggcttgatcggccttcttgcgcatctcacgcgctcctgcggcggcctgtagggcaggctcatacccctgccgaaccgcttttgtcagccggtcggccacggcttccggcgtctcaacgcgctttgagattcccagcttttcggccaatccctgcggtgcataggcgcgtggctcgaccgcttgcgggctgatggtgacgtggcccactggtggccgctccagggcctcgtagaacgcctgaatgcgcgtgtgacgtgccttgctgccctcgatgccccgttgcagccctagatcggccacagcggccgcaaacgtggtctggtcgcgggtcatctgcgctttgttgccgatgaactccttggccgacagcctgccgtcctgcgtcagcggcaccacgaacgcggtcatgtgcgggctggtttcgtcacggtggatgctggccgtcacgatgcgatccgccccgtacttgtccgccagccacttgtgcgccttctcgaagaacgccgcctgctgttcttggctggccgacttccaccattccgggctggccgtcatgacgtactcgaccgccaacacagcgtccttgcgccgcttctctggcagcaactcgcgcagtcggcccatcgcttcatcggtgctgctggccgcccagtgctcgttctctggcgtcctgctggcgtcagcgttgggcgtctcgcgctcgcggtaggcgtgcttgagactggccgccacgttgcccattttcgccagcttcttgcatcgcatgatcgcgtatgccgccatgcctgcccctcccttttggtgtccaaccggctcgacgggggcagcgcaaggcggtgcctccggcgggccactcaatgcttgagtatactcactagactttgcttcgcaaagtcgtgaccgcctacggcggctgcggcgccctacgggcttgctctccgggcttcgccctgcgcggtcgctgcgctcccttgccagcccgtggatatgtggacgatggccgcgagcggccaccggctggctcgcttcgctcggcccgtggacaaccctgctggacaagctgatggacaggctgcgcctgcccacgagcttgaccacagggattgcccaccggctacccagccttcgaccacatacccaccggctccaactgcgcggcctgcggccttgccccatcaatttttttaattttctctggggaaaagcctccggcctgcggcctgcgcgcttcgcttgccggttggacaccaagtggaaggcgggtcaaggctcgcgcagcgaccgcgcagcggcttggccttgacgcgcctggaacgacccaagcctatgcgagtgggggcagtcgaaggcgaagcccgcccgcctgccccccgagcctcacggcggcgagtgcgggggttccaagggggcagcgccaccttgggcaaggccgaaggccgcgcagtcgatcaacaagccccggaggggccactttttgccggagggggagccgcgccgaaggcgtgggggaaccccgcaggggtgcccttctttgggcaccaaagaactagatatagggcgaaatgcgaaagacttaaaaatcaacaacttaaaaaaggggggtacgcaacagctcattgcggcaccccccgcaatagctcattgcgtaggttaaagaaaatctgtaattgactgccacttttacgcaacgcataattgttgtcgcgctgccgaaaagttgcagctgattgcgcatggtgccgcaaccgtgcggcaccctaccgcatggagataagcatggccacgcagtccagagaaatcggcattcaagccaagaacaagcccggtcactgggtgcaaacggaacgcaaagcgcatgaggcgtgggccgggcttattgcgaggaaacccacggcggcaatgctgctgcatcacctcgtggcgcagatgggccaccagaacgccgtggtggtcagccagaagacactttccaagctcatcggacgttctttgcggacggtccaatacgcagtcaaggacttggtggccgagcgctggatctccgtcgtgaagctcaacggccccggcaccgtgtcggcctacgtggtcaatgaccgcgtggcgtggggccagccccgcgaccagttgcgcctgtcggtgttcagtgccgccgtggtggttgatcacgacgaccaggacgaatcgctgttggggcatggcgacctgcgccgcatcccgaccctgtatccgggcgagcagcaactaccgaccggccccggcgaggagccgcccagccagcccggcattccgggcatggaaccagacctgccagccttgaccgaaacggaggaatgggaacggcgcgggcagcagcgcctgccgatgcccgatgagccgtgttttctggacgatggcgagccgttggagccgccgacacgggtcacgctgccgcgccggtagcacttgggttgcgcagcaacccgtaagtgcgctgttccagactatcggctgtagccgcctcgccgccctataccttgtctgcctccccgcgttgcgtcgcggtgcatggagccgggccacctcgacctgaatggaagccggcggcacctcgctaacggattcaccgtttttatcaggctctgggaggcagaataaatgatcatatcgtcaattattacctccacggggagagcctgagcaaactggcctcaggcatttgagaagcacacggtcacactgcttccggtagtcaataaaccggtaaaccagcaatagacataagcggctatttaacgaccctgccctgaaccgacgaccgggtcgaatttgctttcgaatttctgccattcatccgcttattatcacttattcaggcgtagcaccaggcgtttaagggcaccaataactgccttaaaaaaattacgccccgccctgccactcatcgcagtcggcctattggttaaaaaatgagctgatttaacaaaaatttaacgcgaattttaacaaaatattaacgcttacaatttccattcgccattcaggctgcgcaactgttgggaagggcgatcggtgcgggcctcttcgctattacgccagctggcgaaagggggatgtgctgcaaggcgattaagttgggtaacgccagggttttcccagtcacgacgttgtaaaacgacggccagtgagcgcgcgtaatacgactcactatagggcgaattggagctccaccgcggtggcggccgctctagaactagtggatcccccgggctgcaggaattcgatatcaagcttatcgataccgtcgacctcgagttaagtctctaatcgattgttttccaatggaatggttataaaatctttggtttttagtcttgaaaatcttctaggattttctatgtaagtttttgtataaatattatattgctttaataaatttaatatatttttattgcattttaaggttattttttccatatctgttcaaccttttttaaatcctccaaacagtcaatatctaaacttgagctttcgtccattaaaaaatgcttggttttgctttgtaaaaagctaggattgtttaaaaattcttttatctttaaaatataaattgcaccattgctcatataagttttaggcaatttttgccttggcataaaaggatattcatcattacaaatccctgctaaatcgccacaatcattacaaacaaaggcttttagaattttattatcacattcgcttacgctaattagggcatttgcattgctatttttataaagattaaaagcttcattaatatgaatatttgttcttagcggtgaagtgggttgtaaaaaaactacatcttcataatctttataaaattttagagcatgtaacagcactttatcgcttgtggtatcatcttgtgcaaggctaattgggcgttttaaaatatcaacattttgactttttgcataatttaaaatttcatcactatcactgcttacaacaactttactaatgcttttagcatttagtgcagctttgatcgtgtagtaaattaaaggtttattgtttaataaaaccaaatttttatttttaataccctttgagccaccacgagcagggattattgctaagctcattttatatccttaaaaactttttgtgtgctgagtttaaaaaaatctccgctttgtaaatattcaaaaaataattttgagctatctaaaatctctaacttagcgctaaataaatcttgttttttatgaatagtgttaatagcttttagtatttcatcactatttgcattaacttttagtgtattttcattgccaagtcttccattttgtcttgagccaactaaaatccctgctgtttttaagtataaggcctcttttaaaatacaacttgaattacctattataaaatcagcattttttaacaaagttataaaatactcaaatctaagcgatggaaaaagcttaaatctagggttatttttaaactcttcatagctttgcaagattaattcaaaacctaaatcattatttggataaataacaatataatttttattactttgtatcagtgcttttactaaattgtctgcttgatttttaatgctagtaatttcagttgtaacaggatgaaacataagcaaagcgtagttttcataatttatatcataatatttttttgcttcgctaagtgaaattttattatcgtttaaaagttctaaatcaggcgaacctatgataaaaatagatttttcatcttctccaagctgcattaaacgcctttttgcaaactcatcatttactaaatgaatatgagctagttttgatatagcgtggcgtaagctatcgtcaatagttcctgaaatctctccgccttcaatatgcgctactaagatattatttaatgctccaacaatagctgctgctaaaggctcaattctatctccatgtactacgattaaatcaggttttagctcatttgcataccttgaaaatccatcaattgtagtagctaaagccttatcagtttgataatatttatcataatttataaattcataaatatttttaaagccatttttataaagttctttaactgtatagccaaaatttttacttaagtgcattcctgttgcaaagatgtaaagttcaaattcgcttgagttttgcaccctgtacattaaagatttaatcttagaataatcagccctagagcctgttataaaaaggatttttttcacgcaaaatcctcatagcttaactgagcatcattttctatatctcttaatgcttttttgcctaaaatattttcaaattcagccgcactaattccaccaagtccaggtcttttaacccaaatattatccatagataaaacttcgccttttttaatatctttaatgctaactacacttgcaaaggcaaaatcaattgtaacttgttcttgtttagccgcttttttactttcattatttcctcttattatagccatttgctcactttgtataattagctcttttaaagcctttgtatccatagaacaaactatatcagggccacttctatgcatactatcagtaaaatgtctttcaagcacacaagctccaagtacaactgcacctaaacacgcaagattatctgttgtgtggtcgcttaagcctaccatacaagaaaattctttttttaactcaagcatagcgtttaatcttacaagattatgcggggttgggtaaagattggtcgtgtgcattaaaacaaaaggaatttcattgtctaataagatttttacagttggttttatactttcaatactattcattcctgtgctaactatcataggctttttaaaggctgctatgtgtttaataagcggataattattacactcacctgaaccaatcttaaaagcactaactcccatatcttctaagcggttcgcacctgcacgagaaaaaggtgtgctaagataaacaagacctaatttttctgtgtattctttaagtgctagctcatctttataatccaaagcacatttttgcataatctcataaatgcttatttttgcattaccaggaattacttttttagcggccttactcatctcatcttcaacaatatgagtttgatgctttataatcttagcacctgcgctaaaggctgcatctaccataattttagctagttctaaactgccattatgattaatgcctatttcaggtacgactaagggtgctttttcttcacttatgattatattttgtatttttatttctttcatttattttcctccttag

SEQ ID NO: 6 - DNA, 4426 bp, synthetic construct
  misc_feature 1..4426: note = engineered plasmid
  source 1..4426: mol_type = other DNA
ctaaattgtaagcgttaatattttgttaaaattcgcgttaaatttttgttaaatcagctcattttttaaccaataggccgaaatcggcaaaatcccttataaatcaaaagaatagaccgagatagggttgagtgttgttccagtttggaacaagagtccactattaaagaacgtggactccaacgtcaaagggcgaaaaaccgtctatcagggcgatggcccactacgtgaaccatcaccctaatcaagttttttggggtcgaggtgccgtaaagcactaaatcggaaccctaaagggagcccccgatttagagcttgacggggaaagccggcgaacgtggcgagaaaggaagggaagaaagcgaaaggagcgggcgctagggcgctggcaagtgtagcggtcacgctgcgcgtaaccaccacacccgccgcgcttaatgcgccgctacagggcgcgtcccattcgccattcaggctgcgcaactgttgggaagggcgatcggtgcgggcctcttcgctattacgccagctggcgaaagggggatgtgctgcaaggcgattaagttgggtaacgccagggttttcccagtcacgacgttgtaaaacgacggccagtgagcgcgcgtaatacgactcactatagggcgaattggagctccaccgcggtggcggccgctctagaactagtggatccctagactgcaatacaaacacctgtttcacaatttggcagatcagcccaaaaaagtacattctcttcttttacaatacctagttttatcattacttgaactaaaggacttctcaaagcagtttcacgatcagttatagtttctgtcgatgtaaaaactataaatttaattttttcagctggtatcgtgaaatataaagagctcgctataccagcaactgcatcaggaagcatatctgtcatcatcaaaacttcaaatgatatttttgatggaatatcaaccattgaaggatagttttgcattattaatgtattaatgataccgccaccagggtgacctttgaagaacaaatcataactattgcctaaataatgtgggctcgattcattaattgcattattaatgacattaatttgttgtttcgcataatactctctttcatggttaccagcccatacagtcgtacctgtaaacacaaagtttggtaaattagatgaattatattcattttgtaatttttgtttgtcaaaattaacaatcgataagaataattcttgttgtttgctattgaattttttgaaaccatcccattgcatttgctttaaactatcaccaatatagtctcgtaactcatgtaatgatggttctaaagttaaataatcttttcttaaaaaatggtagttagctggatatagtttttgccagttataaacagatgatgttcctgtatttgaagtgtcttcattgataccattaatgacatcctcaagataatctttaccaatttttaaattatctgttttatttaatgtatctctccagttatataaatttacatattctgctgaaccatcatcatataaatctatatttgttaccgtaacgttattaaacgaatttaattcttttagtattggcactaaattatcaaatgaatgagcagtgttagagctaagtttaacattcaatctatgctttgtttgtgcttgcttaacaatttcttgtactaagtcagctggtgtatggttatttatcaatgcaaacgatgtaatatttaactctttcatttgctcatcagtcggaactattctcccccaagctatatatctttgtgctgtaggattttcttcttccgatttaataatatccattagctgctgaagagttggaagagatgcatgatcaacataaacctctaaagatggagccactacgtttaatgttacttttgttatatatttttcacctttattactaacaccattaaaatcaaagcagtacttttcatcgtcatctaatcgtggcgccactacagataatgatattgactctttattttgttctgttaatagttgttgcgtaccacaagtttgtacccaagagtgttttgtaaaagagatgtttgattgattaattggctctaaattaacatactcctcatcaataatagttttattaatatcatttttaataatagattgtgtattttcttctgacatggtctgtttcctcctcgagggggggcccggtacccagcttttgttccctttagtgagggttaattgcgcgcttggcgtaatcatggtcatagctgtttcctgtgtgaaattgttatccgctcacaattccacacaacatacgagccggaagcataaagtgtaaagcctggggtgcctaatgagtgagctaactcacattaattgcgttgcgctcactgcccgctttccagtcgggaaacctgtcgtgccagctgcattaatgaatcggccaacgcgcggggagaggcggtttgcgtattgggcgctcttccgcttcctcgctcactgactcgctgcgctcggtcgttcggctgcggcgagcggtatcagctcactcaaaggcggtaatacggttatccacagaatcaggggataacgcaggaaagaacatgtgagcaaaaggccagcaaaaggccaggaaccgtaaaaaggccgcgttgctggcgtttttccataggctccgcccccctgacgagcatcacaaaaatcgacgctcaagtcagaggtggcgaaacccgacaggactataaagataccaggcgtttccccctggaagctccctcgtgcgctctcctgttccgaccctgccgcttaccggatacctgtccgcctttctcccttcgggaagcgtggcgctttctcatagctcacgctgtaggtatctcagttcggtgtaggtcgttcgctccaagctgggctgtgtgcacgaaccccccgttcagcccgaccgctgcgccttatccggtaactatcgtcttgagtccaacccggtaagacacgacttatcgccactggcagcagccactggtaacaggattagcagagcgaggtatgtaggcggtgctacagagttcttgaagtggtggcctaactacggctacactagaaggacagtatttggtatctgcgctctgctgaagccagttaccttcggaaaaagagttggtagctcttgatccggcaaacaaaccaccgctggtagcggtggtttttttgtttgcaagcagcagattacgcgcagaaaaaaaggatctcaagaagatcctttgatcttttctacggggtctgacgctcagtggaacgaaaactcacgttaagggattttggtcatgagattatcaaaaaggatcttcacctagatccttttaaattaaaaatgaagttttaaatcaatctaaagtatatatgagtaaacttggtctgacagttaccaatgcttaatcagtgaggcacctatctcagcgatctgtctatttcgttcatccatagttgcctgactccccgtcgtgtagataactacgatacgggagggcttaccatctggccccagtgctgcaatgataccgcgagacccacgctcaccggctccagatttatcagcaataaaccagccagccggaagggccgagcgcagaagtggtcctgcaactttatccgcctccatccagtctattaattgttgccgggaagctagagtaagtagttcgccagttaatagtttgcgcaacgttgttgccattgctacaggcatcgtggtgtcacgctcgtcgtttggtatggcttcattcagctccggttcccaacgatcaaggcgagttacatgatcccccatgttgtgcaaaaaagcggttagctccttcggtcctccgatcgttgtcagaagtaagttggccgcagtgttatcactcatggttatggcagcactgcataattctcttactgtcatgccatccgtaagatgcttttctgtgactggtgagtactcaaccaagtcattctgagaatagtgtatgcggcgaccgagttgctcttgcccggcgtcaatacgggataataccgcgccacatagcagaactttaaaagtgctcatcattggaaaacgttcttcggggcgaaaactctcaaggatcttaccgctgttgagatccagttcgatgtaacccactcgtgcacccaactgatcttcagcatcttttactttcaccagcgtttctgggtgagcaaaaacaggaaggcaaaatgccgcaaaaaagggaataagggcgacacggaaatgttgaatactcatactcttcctttttcaatattattgaagcatttatcagggttattgtctcatgagcggatacatatttgaatgtatttagaaaaataaacaaataggggttccgcgcacatttccccgaaaagtgccac

SEQ ID NO: 7 - DNA, 22 bp, synthetic construct
  misc_feature 1..22: note = chemically synthesized oligonucleotide
  source 1..22: mol_type = other DNA
ctcgaggaggaaacagaccatg

SEQ ID NO: 8 - DNA, 28 bp, synthetic construct
  misc_feature 1..28: note = chemically synthesized oligonucleotide
  source 1..28: mol_type = other DNA
ctcgaggaaagaggggacaaactagatg

SEQ ID NO: 9 - DNA, 4432 bp, synthetic construct
  misc_feature 1..4432: note = engineered plasmid
  source 1..4432: mol_type = other DNA
ctaaattgtaagcgttaatattttgttaaaattcgcgttaaatttttgttaaatcagctcattttttaaccaataggccgaaatcggcaaaatcccttataaatcaaaagaatagaccgagatagggttgagtgttgttccagtttggaacaagagtccactattaaagaacgtggactccaacgtcaaagggcgaaaaaccgtctatcagggcgatggcccactacgtgaaccatcaccctaatcaagttttttggggtcgaggtgccgtaaagcactaaatcggaaccctaaagggagcccccgatttagagcttgacggggaaagccggcgaacgtggcgagaaaggaagggaagaaagcgaaaggagcgggcgctagggcgctggcaagtgtagcggtcacgctgcgcgtaaccaccacacccgccgcgcttaatgcgccgctacagggcgcgtcccattcgccattcaggctgcgcaactgttgggaagggcgatcggtgcgggcctcttcgctattacgccagctggcgaaagggggatgtgctgcaaggcgattaagttgggtaacgccagggttttcccagtcacgacgttgtaaaacgacggccagtgagcgcgcgtaatacgactcactatagggcgaattggagctccaccgcggtggcggccgctctagaactagtggatccctagactgcaatacaaacacctgtttcacaatttggcagatcagcccaaaaaagtacattctcttcttttacaatacctagttttatcattacttgaactaaaggacttctcaaagcagtttcacgatcagttatagtttctgtcgatgtaaaaactataaatttaattttttcagctggtatcgtgaaatataaagagctcgctataccagcaactgcatcaggaagcatatctgtcatcatcaaaacttcaaatgatatttttgatggaatatcaaccattgaaggatagttttgcattattaatgtattaatgataccgccaccagggtgacctttgaagaacaaatcataactattgcctaaataatgtgggctcgattcattaattgcattattaatgacattaatttgttgtttcgcataatactctctttcatggttaccagcccatacagtcgtacctgtaaacacaaagtttggtaaattagatgaattatattcattttgtaatttttgtttgtcaaaattaacaatcgataagaataattcttgttgtttgctattgaattttttgaaaccatcccattgcatttgctttaaactatcaccaatatagtctcgtaactcatgtaatgatggttctaaagttaaataatcttttcttaaaaaatggtagttagctggatatagtttttgccagttataaacagatgatgttcctgtatttgaagtgtcttcattgataccattaatgacatcctcaagataatctttaccaatttttaaattatctgttttatttaatgtatctctccagttatataaatttacatattctgctgaaccatcatcatataaatctatatttgttaccgtaacgttattaaacgaatttaattcttttagtattggcactaaattatcaaatgaatgagcagtgttagagctaagtttaacattcaatctatgctttgtttgtgcttgcttaacaatttcttgtactaagtcagctggtgtatggttatttatcaatgcaaacgatgtaatatttaactctttcatttgctcatcagtcggaactattctcccccaagctatatatctttgtgctgtaggattttcttcttccgatttaataatatccattagctgctgaagagttggaagagatgcatgatcaacataaacctctaaagatggagccactacgtttaatgttacttttgttatatatttttcacctttattactaacaccattaaaatcaaagcagtacttttcatcgtcatctaatcgtggcgccactacagataatgatattgactctttattttgttctgttaatagttgttgcgtaccacaagtttgtacccaagagtgttttgtaaaagagatgtttgattgattaattggctctaaattaacatactcctcatcaataatagttttattaatatcatttttaataatagattgtgtattttcttctgacatctagtttgtcccctctttcctcgagggggggcccggtacccagcttttgttccctttagtgagggttaattgcgcgcttggcgtaatcatggtcatagctgtttcctgtgtgaaattgttatccgctcacaattccacacaacatacgagccggaagcataaagtgtaaagcctggggtgcctaatgagtgagctaactcacattaattgcgttgcgctcactgcccgctttccagtcgggaaacctgtcgtgccagctgcattaatgaatcggccaacgcgcggggagaggcggtttgcgtattgggcgctcttccgcttcctcgctcactgactcgctgcgctcggtcgttcggctgcggcgagcggtatcagctcactcaaaggcggtaatacggttatccacagaatcaggggataacgcaggaaagaacatgtgagcaaaaggccagcaaaaggccaggaaccgtaaaaaggccgcgttgctggcgtttttccataggctccgcccccctgacgagcatcacaaaaatcgacgctcaagtcagaggtggcgaaacccgacaggactataaagataccaggcgtttccccctggaagctccctcgtgcgctctcctgttccgaccctgccgcttaccggatacctgtccgcctttctcccttcgggaagcgtggcgctttctcatagctcacgctgtaggtatctcagttcggtgtaggtcgttcgctccaagctgggctgtgtgcacgaaccccccgttcagcccgaccgctgcgccttatccggtaactatcgtcttgagtccaacccggtaagacacgacttatcgccactggcagcagccactggtaacaggattagcagagcgaggtatgtaggcggtgctacagagttcttgaagtggtggcctaactacggctacactagaaggacagtatttggtatctgcgctctgctgaagccagttaccttcggaaaaagagttggtagctcttgatccggcaaacaaaccaccgctggtagcggtggtttttttgtttgcaagcagcagattacgcgcagaaaaaaaggatctcaagaagatcctttgatcttttctacggggtctgacgctcagtggaacgaaaactcacgttaagggattttggtcatgagattatcaaaaaggatcttcacctagatccttttaaattaaaaatgaagttttaaatcaatctaaagtatatatgagtaaacttggtctgacagttaccaatgcttaatcagtgaggcacctatctcagcgatctgtctatttcgttcatccatagttgcctgactccccgtcgtgtagataactacgatacgggagggcttaccatctggccccagtgctgcaatgataccgcgagacccacgctcaccggctccagatttatcagcaataaaccagccagccggaagggccgagcgcagaagtggtcctgcaactttatccgcctccatccagtctattaattgttgccgggaagctagagtaagtagttcgccagttaatagtttgcgcaacgttgttgccattgctacaggcatcgtggtgtcacgctcgtcgtttggtatggcttcattcagctccggttcccaacgatcaaggcgagttacatgatcccccatgttgtgcaaaaaagcggttagctccttcggtcctccgatcgttgtcagaagtaagttggccgcagtgttatcactcatggttatggcagcactgcataattctcttactgtcatgccatccgtaagatgcttttctgtgactggtgagtactcaaccaagtcattctgagaatagtgtatgcggcgaccgagttgctcttgcccggcgtcaatacgggataataccgcgccacatagcagaactttaaaagtgctcatcattggaaaacgttcttcggggcgaaaactctcaaggatcttaccgctgttgagatccagttcgatgtaacccactcgtgcacccaactgatcttcagcatcttttactttcaccagcgtttctgggtgagcaaaaacaggaaggcaaaatgccgcaaaaaagggaataagggcgacacggaaatgttgaatactcatactcttcctttttcaatattattgaagcatttatcagggttattgtctcatgagcggatacatatttgaatgtatttagaaaaataaacaaataggggttccgcgcacatttccccgaaaagtgccac

SEQ ID NO: 10 - DNA, 19 bp, synthetic construct
  misc_feature 1..19: note = chemically synthesized oligonucleotide
  source 1..19: mol_type = other DNA
ctttattaaacctactatg

SEQ ID NO: 11 - DNA, 19 bp, synthetic construct
  misc_feature 1..19: note = chemically synthesized oligonucleotide
  source 1..19: mol_type = other DNA
ctttcttcaacctactatg

SEQ ID NO: 12 - DNA, 7916 bp, synthetic construct
  misc_feature 1..7916: note = engineered plasmid
  source 1..7916: mol_type = other DNA
tcgcgcgtttcggtgatgacggtgaaaacctctgacacatgcagctcccggagacggtcacagcttgtctgtaagcggatgccgggagcagacaagcccgtcagggcgcgtcagcgggtgttggcgggtgtcggggctggcttaactatgcggcatcagagcagattgtactgagagtgcaccatatatgcggtgtgaaataccgcacagatgcgtaaggagaaaataccgcatcaggcgccactagtgttgaggaaaacgattggctgaacaaaaaacagactgatcgaggtcatttttgagtgcaaaaagtgctgtaactctgaaaaagcgatggtagaatccatttttaagcaaacggtgattttgaaaaatgggtaacaacgtcgtcgtactgggcacccaatggggtgacgaaggtaaaggtaagatcgtcgatcttctgactgaacgggctaaatatgttgtacgctaccagggcggtcacaacgcaggccatactctcgtaatcaacggtgaaaaaaccgttctccatcttattccatcaggtattctccgcgagaatgtaaccagcatcatcggtaacggtgttgtgctgtctccggccgcgctgatgaaagagatgaaagaactggaagaccgtggcatccccgttcgtgagcgtctgctgctgtctgaagcatgtccgctgatccttgattatcacgttgcgctggataacgcgcgtgagaaagcgcgtggcgcgaaagcgatcggcaccaccggtcgtggtatcgggcctgcttatgaagataaagtagcacgtcgcggtctgcgtgttggcgaccttttcgacaaagaaaccttcgctgaaaaactgaaagaagtgatggaatatcacaacttccagttggttaactactacaaagctgaagcggttgattaccagaaagttctggatgatacgatggctgttgccgacatcctgacttctatggtggttgacgtttctgacctgctcgaccaggcgcgtcagcgtggcgatttcgtcatgtttgaaggtgcgcagggtacgctgctggatatcgaccacggtacttatccgtacgtaacttcttccaacaccactgctggtggcgtggcgaccggttccggcctgggcccgcgttatgttgattacgttctgggtatcctcaaagcttactccactcgtgtaggtgcaggtccgttcccgaccgaactgtttgatgaaactggcgagttcctctgcaagcagggtaacgaattcggcgcaactacggggcgtcgtcgtcgtaccggctggctggacaccgttgccgttcgtcgtgcggtacagctgaactccctgtctggcttctgcctgactaaactggacgttctggatggcctgaaagaggttaaactctgcgtggcttaccgtatgccggatggtcgcgaagtgactaccactccgctggcagctgacgactggaaaggtgtagagccgatttacgaaaccatgccgggctggtctgaatccaccttcggcgtgaaagatcgtagcggcctgccgcaggcggcgctgaactatatcaagcgtattgaagagctgactggtgtgccgatcgatatcatctctaccggtccggatcgtactgaaaccatgattctgcgcgacccgttcgacgcgtaattctggtacgcctggcagatattttgcctgccgggcgaacagtgtgatacattgctgtgtcgggtaagccattacgctatccgacacagtgttaaatcctcgcttttttccttccccagatctggcgccattcgccattcaggctgcgcaactgttgggaagggcgatcggtgcgggcctcttcgctattacgccagctggcgaaagggggatgtgctgcaaggcgattaagttgggtaacgccagggttttcccagtcacgacgttgtaaaacgacggccagtgccaagcttactgctcacaagaaaaaaggcacgtcatctgacgtgccttttttatttgtactaccctgtacgattactgcaggtcgacttaattttccagcaaatgctggagcaaaataccgttgagcatggcgcgttttaccagcgcaaaagcgccgattgccgagcggtgatccagctcagaacgtaccaccggcagattagtgcgaaacgccttcagcgcctgggtattaatgcagctttcaatagcagggagcagcactttatcggcttcggtgatttcaccggcaataacaattttttgcggattaaataagttgatagcaatggcgatggttttacccagatgacgaccgacatactcaattacttccgacgccagactatcgcctttgttcgcggctttgcagatagttttgatggtgcagtcgtccagcggcacgcggctctggtagccctgctttaacagattcaacacccgttgttcaatggcagcgttggcagcgatagtttccaggcagccaaagttgccgcagtggcagcgttcacccagcggttcgacctgaatatggccaatttcaccgacgttgccgttgcggccaataaaaatgcgcccgttagagataatcccggccccggttccgcgatggacacgcaccagaatggagtcttcgcaatcctgacttgcaccgaagtagtgctccgccagcgccagactacggatatcgtgaccaacgaaacaggtcactttaaaacgttcttccagagcttctaccagcccccagttttctacctgaatatgcggcatgtaatgaattttgccgctgtccgggtcaacaagccctggcaggatcaccgaaatcgcgatcagctcgcgcagtttgcgctggtagctatcaataaactgagcaatggcattcaacagggcatgttccagcgtttgctgggtacgttccggcagcgggtaatgttcttctgccagcactttgctgctgagatcaaacagagtgatggtggcgtcatgacgaccaagccgtacgccgattgcgtggaaattgcgggtttcggtgacgatggagatagcgcggcggcccccggtggaggcctgctgatcaacttctttgatcagcccgcgttcgataagctgacgcgtaattttggttacgctggcgggggcaagctggctttgctcggcaatctgaatccgcgagattggcccgtactggtcaatcaggcgataaaccgccgcgctgttaagctgttttacgagatcaacattacctatctgagcttgtccgcctggtgtcatatgtatatctccttcttgtcgactctagatgcatgctcgagattactcaaccgtaaccgattttgccaggttacgcggctggtcaacgtcggtgcctttgatcagcgcgacatggtaagccagcagctgcagcggaacggtgtagaagatcggtgcaatcacctcttccacatgcggcatctcgatgatgtgcatgttatcgctacttacaaaacccgcatcctgatcggcgaagacatacaactgaccgccacgcgcgcgaacttcttcaatgttggatttcagtttttccagcaattcgttgttcggtgcaacaacaataaccggcatatcggcatcaattagcgccagcggaccgtgtttcagttcgccagcagcgtaggcttcagcgtgaatgtaagagatctctttcaacttcaatgcgccttccagcgcgattgggtactgatcgccacggcccaggaacagcgcgtgatgtttgtcagagaaatcttctgccagcgcttcaatgcgtttgtcctgagacagcatctgctcaatacggctcggcagcgcctgcagaccatgcacgatgtcatgttcaatggaggcatccagacctttcaggcgagacagcttcgccaccagcatcaacagcacagttaactgagtggtgaatgctttagtggatgccacgccgatttctgtacccgcgttggtcattagcgccagatcggattcgcgcaccagagaagaacccggaacgttacagattgccagtgaaccaaggtaacccagctctttcgacagacgcaggccagccagggtatccgcggtttcgccagactgtgacaaggtgatcatcaggctgttacgacgcacggcagatttgcgatagcggaattcagaggcgatttcgacgtcgcacggaatacctgctagcgattcaaaccagtagcgggaaaccataccggagttataagaagtaccacaggcgaggatctgaatatgctcaaccttcgacagcagttcgtcggcgttcggtcccagctcgcttaaatcaacctgaccgtggctgatgcgtccggtaagggtgtttttgatcgcgttcggctgttcgtagatctctttctgcatgtagtgacggtaaatgcctttatcgcccgcgtcatattgcagattggattcgatatcctgacgttttacttccgcgccagttttatcgaagatgtttaccgaacggcgagtgatttccgcaatatcgccctcttcaaggaagataaagcgacgggtcaccggcaacagcgccagctggtcagaagcgataaagttttcgcccatccccaggccaatcaccagcggactaccagaacgtgccgccagcagggtatccgggtgacgggagtccatgatcactgtaccgtacgcaccacgcagctgcgggatagcacgcagaacggcctcacgcagagtcccgccttgtttcagctcccagttcaccagatgggcaatcacttcggtgtcggtttcagaaacgaaggtatagccacgcgcttttagctcttcacgcagcggttcatggttttcgatgatgccgttatgcaccaccacaatgtgttcagaaacatgcggatgcgcattcacttctgaaggttcaccgtgggtcgcccagcgagtgtgagcaataccagtgccgccatgcagaggatgttcttccgctgcctgtgccagcatctggactttaccgaggcgacgcaggcgggtcatatgaccttctgcatcaacaacggccagaccggcagagtcatatccgcggtattccagacgacgtaaaccttcaagaaggatttctgctacatcacgttgcgcgatcgcgccaacaattccacacatatgtatatctccttcttgaattctaacaattgattgaatgtatgcaaataaatgcatacaccataggtgtggtttaatttgatgccctttttcagggctggaatgtgtaagagcggggttatttatgctgttgtttttttgttactcgggaagggctttacctcttccgcataaacgcttccatcagcgtttatagttaaaaaaatctttcggaactggttttgcgcttaccccaaccaacaggggatttgctgctttccattgagcctgtttctctgcgcgacgttcgcggcggcgtgtttgtgcatccatctggattctcctgtcagttagctttggtggtgtgtggcagttgtagtcctgaacgaaaaccccccgcgattggcacattggcagctaatccggaatcgcacttacggccaatgcttcgtttcgtatcacacaccccaaagccttctgctttgaatgctgcccttcttcagggcttaatttttaagagcgtcaccttcatggtggtcagtgcgtcctgctgatgtgctcagtatcaccgccagtggtatttatgtcaacaccgccagagataatttatcaccgcagatggttatctgtatgttttttatatgaatttattttttgcaggggggcattgtttggtaggtgagagatcaattctgcattaatgaatcggccaacgcgcggggagaggcggtttgcgtattgggcgctcttccgctgctagcggagtgtatactggcttactatgttggcactgatgagggtgtcagtgaagtgcttcatgtggcaggagaaaaaaggctgcaccggtgcgtcagcagaatatgtgatacaggatatattccgcttcctcgctcactgactcgctacgctcggtcgttcgactgcggcgagcggaaatggcttacgaacggggcggagatttcctggaagatgccaggaagatacttaacagggaagtgagagggccgcggcaaagccgtttttccataggctccgcccccctgacaagcatcacgaaatctgacgctcaaatcagtggtggcgaaacccgacaggactataaagataccaggcgtttccccctggcggctccctcgtgcgctctcctgttcctgcctttcggtttaccggtgtcattccgctgttatggccgcgtttgtctcattccacgcctgacactcagttccgggtaggcagttcgctccaagctggactgtatgcacgaaccccccgttcagtccgaccgctgcgccttatccggtaactatcgtcttgagtccaacccggaaagacatgcaaaagcaccactggcagcagccactggtaattgatttagaggagttagtcttgaagtcatgcgccggttaaggctaaactgaaaggacaagttttggtgactgcgctcctccaagccagttacctcggttcaaagagttggtagctcagagaaccttcgaaaaaccgccctgcaaggcggttttttcgttttcagagcaagagattacgcgcagaccaaaacgatctcaagaagatcatcttattaatcagataaaatatttctaggcggccgcgaacgaaaactcacgttaagggattttggtcatgagattatcaaaaaggatcttcacctagatccttttaaattaaaaatgaagttttaaatcaatctaaagtatatatgagtaaacttggtctgacagttaccaatgcttaatcagtgaggcacctatctcagcgatctgtctatttcgttcatccatagttgcctgactccccgtcgtgtagataactacgatacgggagggcttaccatctggccccagtgctgcaatgataccgcgagacccacgctcaccggctccagatttatcagcaataaaccagccagccggaagggccgagcgcagaagtggtcctgcaactttatccgcctccatccagtctattaattgttgccgggaagctagagtaagtagttcgccagttaatagtttgcgcaacgttgttgccattgctacaggcatcgtggtgtcacgctcgtcgtttggtatggcttcattcagctccggttcccaacgatcaaggcgagttacatgatcccccatgttgtgcaaaaaagcggttagctccttcggtcctccgatcgttgtcagaagtaagttggccgcagtgttatcactcatggttatggcagcactgcataattctcttactgtcatgccatccgtaagatgcttttctgtgactggtgagtactcaaccaagtcattctgagaatagtgtatgcggcgaccgagttgctcttgcccggcgtcaatacgggataataccgcgccacatagcagaactttaaaagtgctcatcattggaaaacgttcttcggggcgaaaactctcaaggatcttaccgctgttgagatccagttcgatgtaacccactcgtgcacccaactgatcttcagcatcttttactttcaccagcgtttctgggtgagcaaaaacaggaaggcaaaatgccgcaaaaaagggaataagggcgacacggaaatgttgaatactcatactcttcctttttcaatattattgaagcatttatcagggttattgtctcatgagcggatacatatttgaatgtatttagaaaaataaacaaataggggttccgcgcacatttccccgaaaagtgccacctgacgtctaagaaaccattattatcatgacattaacctataaaaataggcgtatcacgaggccctttcgtc

SEQ ID NO: 13 - protein, 372 aa, Campylobacter jejuni
MKKILFITGSRADYSKIKSLMYRVQNSSEFELYIFATGMHLSKNFGYTVKELYKNGFKNIYEFINYDKYYQTDKALATTIDGFSRYANELKPDLIVVHGDRIEPLAAAIVGALNNILVAHIEGGEISGTIDDSLRHAISKLAHIHLVNDEFAKRRLMQLGEDEKSIFIIGSPDLELLNDNKISLSEAKKYYDINYENYALLMFHPVTTEITSIKNQADNLVKALIQSNKNYIVIYPNNDLGFELILQSYEEFKNNPRFKLFPSLRFEYFITLLKNADFIIGNSSCILKEALYLKTAGILVGSRQNGRLGNENTLKVNANSDEILKAINTIHKKQDLFSAKLEILDSSKLFFEYLQSGDFFKLSTQKVFKDIK

SEQ ID NO: 14 - protein, 346 aa, Campylobacter jejuni
MKEIKIQNIIISEEKAPLVVPEIGINHNGSLELAKIMVDAAFSAGAKIIKHQTHIVEDEMSKAAKKVIPGNAKISIYEIMQKCALDYKDELALKEYTEKLGLVYLSTPFSRAGANRLEDMGVSAFKIGSGECNNYPLIKHIAAFKKPMIVSTGMNSIESIKPTVKILLDNEIPFVLMHTTNLYPTPHNLVRLNAMLELKKEFSCMVGLSDHTTDNLACLGAVVLGACVLERHFTDSMHRSGPDIVCSMDTKALKELIIQSEQMAIIRGNNESKKAAKQEQVTIDFAFASVVSIKDIKKGEVLSMDNIWVKRPGLGGISAAEFENILGKKALRDIENDAQLSYEDFA

SEQ ID NO: 15 - protein, 221 aa, Campylobacter jejuni
MSLAIIPARGGSKGIKNKNLVLLNNKPLIYYTIKAALNAKSISKVVVSSDSDEILNYAKSQNVDILKRPISLAQDDTTSDKVLLHALKFYKDYEDVVFLQPTSPLRTNIHINEAFNLYKNSNANALISVSECDNKILKAFVCNDCGDLAGICNDEYPFMPRQKLPKTYMSNGAIYILKIKEFLNNPSFLQSKTKHFLMDESSSLDIDCLEDLKKVEQIWKK

SEQ ID NO: 16 - protein, 349 aa, Neisseria meningitidis
MPSEAFRRHRAYRENKLQPLVSVLICAYNVEKYFAQSLAAVVNQTWRNLDILIVDDGSTDGTLAIAQRFQEQDGRIRILAQPRNSGLIPSLNIGLDELAKSGGGGEYIARTDADDIAAPDWIEKIVGEMEKDRSIIAMGAWLEVLSEEKDGNRLARHHEHGKIWKKPTRHEDIADFFPFGNPIHNNTMIMRRSVIDGGLRYNTERDWAEDYQFWYDVSKLGRLAYYPEALVKYRLHANQVSSKYSIRQHEIAQGIQKTARNDFLQSMGFKTRFDSLEYRQIKAVAYELLEKHLPEEDFERARRFLYQCFKRTDTLPAGAWLDFAADGRMRRLFTLRQYFGILHRLLKNR

SEQ ID NO: 17 - protein, 273 aa, Helicobacter pylori
MRVFAISLNQKVCDTFGLVFRDTTTLLNSINATHHQAQIFDAIYSKTFEGGLHPLVKKHLHPYFITQNIKDMGITTNLISEVSKFYYALKYHAKFMSLGELGCYASHYSLWEKCIELNEAICILEDDITLKEDFKEGLDFLEKHIQELGYIRLMHLLYDASVKSEPLSHKNHEIQERVGIIKAYSEGVGTQGYVITPKIAKVFLKCSRKWVVPVDTIMDATFIHGVKNLVLQPFVIADDEQISTIARKEEPYSPKIALMRELHFKYLKYWQFV

SEQ ID NO: 18 - protein, 265 aa, Escherichia coli
MIIDEAESAESTHPVVSVILPVNKKNPFLDEAINSILSQTFSSFEIIIVANCCTDDFYNELKHKVNDKIKLIRTNIAYLPYSLNKAIDLSNGEFIARMDSDDISHPDRFTKQVDFLKNNPYVDVVGTNAIFIDDKGREINKTKLPEENLDIVKNLPYKCCIVHPSVMFRKKVIASIGGYMFSNYSEDYELWNRLSLAKIKFQNLPEYLFYYRLHEGQSTAKKNLYMVMVNDLVIKMKCFFLTGNINYLFGGIRTIASFIYCKYIK

SEQ ID NO: 19 - protein, 406 aa, Escherichia coli
MTPGGQAQIGNVDLVKQLNSAAVYRLIDQYGPISRIQIAEQSQLAPASVTKITRQLIERGLIKEVDQQASTGGRRAISIVTETRNFHAIGVRLGRHDATITLFDLSSKVLAEEHYPLPERTQQTLEHALLNAIAQFIDSYQRKLRELIAISVILPGLVDPDSGKIHYMPHIQVENWGLVEALEERFKVTCFVGHDIRSLALAEHYFGASQDCEDSILVRVHRGTGAGIISNGRIFIGRNGNVGEIGHIQVEPLGERCHCGNFGCLETIAANAAIEQRVLNLLKQGYQSRVPLDDCTIKTICKAANKGDSLASEVIEYVGRHLGKTIAIAINLFNPQKIVIAGEITEADKVLLPAIESCINTQALKAFRTNLPVVRSELDHRSAIGAFALVKRAMLNGILLQHLLEN

SEQ ID NO: 20 - protein, 609 aa, Escherichia coli
MCGIVGAIAQRDVAEILLEGLRRLEYRGYDSAGLAVVDAEGHMTRLRRLGKVQMLAQAAEEHPLHGGTGIAHTRWATHGEPSEVNAHPHVSEHIVVVHNGIIENHEPLREELKARGYTFVSETDTEVIAHLVNWELKQGGTLREAVLRAIPQLRGAYGTVIMDSRHPDTLLAARSGSPLVIGLGMGENFIASDQLALLPVTRRFIFLEEGDIAEITRRSVNIFDKTGAEVKRQDIESNLQYDAGDKGIYRHYMQKEIYEQPNAIKNTLTGRISHGQVDLSELGPNADELLSKVEHIQILACGTSYNSGMVSRYWFESLAGIPCDVEIASEFRYRKSAVRRNSLMITLSQSGETADTLAGLRLSKELGYLGSLAICNVPGSSLVRESDLALMTNAGTEIGVASTKAFTTQLTVLLMLVAKLSRLKGLDASIEHDIVHGLQALPSRIEQMLSQDKRIEALAEDFSDKHHALFLGRGDQYPIALEGALKLKEISYIHAEAYAAGELKHGPLALIDADMPVIVVAPNNELLEKLKSNIEEVRARGGQLYVFADQDAGFVSSDNMHIIEMPHVEEVIAPIFYTVPLQLLAYHVALIKGTDVDQPRNLAKSVTVE

SEQ ID NO: 21 - protein, 514 aa, Photobacterium sp. JT-ISH-224
MKNFLLLTLILLTACNNSEENTQSIIKNDINKTIIDEEYVNLEPINQSNISFTKHSWVQTCGTQQLLTEQNKESISLSVVAPRLDDDEKYCFDFNGVSNKGEKYITKVTLNVVAPSLEVYVDHASLPTLQQLMDIIKSEEENPTAQRYIAWGRIVPTDEQMKELNITSFALINNHTPADLVQEIVKQAQTKHRLNVKLSSNTAHSFDNLVPILKELNSFNNVTVTNIDLYDDGSAEYVNLYNWRDTLNKTDNLKIGKDYLEDVINGINEDTSNTGTSSVYNWQKLYPANYHFLRKDYLTLEPSLHELRDYIGDSLKQMQWDGFKKFNSKQQELFLSIVNFDKQKLQNEYNSSNLPNFVFTGTTVWAGNHEREYYAKQQINVINNAINESSPHYLGNSYDLFFKGHPGGGIINTLIMQNYPSMVDIPSKISFEVLMMTDMLPDAVAGIASSLYFTIPAEKIKFIVFTSTETITDRETALRSPLVQVMIKLGIVKEENVLFWADLPNCETGVCIAV

SEQ ID NO: 22 - protein, 156 aa, Escherichia coli
MKTQRGYTLIETLVAMLILVMLSASGLYGWQYWQQSQRLWQTASQARDYLLYLREDANWHNRDHSISVIREGTLWCLVSSAAGANTCHGSSPLVFVPRWPEVEMSDLTPSLAFFGLRNTAWAGHIRFKNSTGEWWLVVSPWGRLRLCQQGETEGCL

SEQ ID NO: 23 - DNA, 37 bp, Escherichia coli
  source 1..37: mol_type = genomic DNA
cagtcagtcaggcgccttcgggaaggcgtctcgaaga

SEQ ID NO: 24 - DNA, 84 bp, Escherichia coli
  source 1..84: mol_type = genomic DNA
ggcgtcggctctggcaggatgtttcgtaattagatagccaccggcgctttaggaaacctactatgaccatgattacggattcac

SEQ ID NO: 25 - DNA, 84 bp, Escherichia coli
  source 1..84: mol_type = genomic DNA
ggcgtcggctctggcaggatgtttcgtaattagatagccaccggcgctttattaaacctactatgaccatgattacggattcac

SEQ ID NO: 26 - DNA, 84 bp, Escherichia coli
  source 1..84: mol_type = genomic DNA
ggcgtcggctctggcaggatgtttcgtaattagatagccaccggcgctttcttcaacctactatgaccatgattacggattcac

SEQ ID NO: 27 - DNA, 84 bp, Escherichia coli; identical to SEQ ID NO: 24
  source 1..84: mol_type = genomic DNA

SEQ ID NO: 28 - DNA, 68 bp, Escherichia coli
  source 1..68: mol_type = genomic DNA
cggctctggcaggatgtttcgtaattagatagccaccggcgctttattaaacctactatgaccatgat

SEQ ID NO: 29 - protein, 1024 aa, Escherichia coli
MTMITDSLAVVLQRRDWENPGVTQLNRLAAHPPFASWRNSEEARTDRPSQQLRSLNGEWRFAWFPAPEAVPESWLECDLPEADTVVVPSNWQMHGYDAPIYTNVTYPITVNPPFVPTENPTGCYSLTFNVDESWLQEGQTRIIFDGVNSAFHLWCNGRWVGYGQDSRLPSEFDLSAFLRAGENRLAVMVLRWSDGSYLEDQDMWRMSGIFRDVSLLHKPTTQISDFHVATRFNDDFSRAVLEAEVQMCGELRDYLRVTVSLWQGETQVASGTAPFGGEIIDERGGYADRVTLRLNVENPKLWSAEIPNLYRAVVELHTADGTLIEAEACDVGFREVRIENGLLLLNGKPLLIRGVNRHEHHPLHGQVMDEQTMVQDILLMKQNNFNAVRCSHYPNHPLWYTLCDRYGLYVVDEANIETHGMVPMNRLTDDPRWLPAMSERVTRMVQRDRNHPSVIIWSLGNESGHGANHDALYRWIKSVDPSRPVQYEGGGADTTATDIICPMYARVDEDQPFPAVPKWSIKKWLSLPGETRPLILCEYAHAMGNSLGGFAKYWQAFRQYPRLQGGFVWDWVDQSLIKYDENGNPWSAYGGDFGDTPNDRQFCMNGLVFADRTPHPALTEAKHQQQFFQFRLSGQTIEVTSEYLFRHSDNELLHWMVALDGKPLASGEVPLDVAPQGKQLIELPELPQPESAGQLWLTVRVVQPNATAWSEAGHISAWQQWRLAENLSVTLPAASHAIPHLTTSEMDFCIELGNKRWQFNRQSGFLSQMWIGDKKQLLTPLRDQFTRAPLDNDIGVSEATRIDPNAWVERWKAAGHYQAEAALLQCTADTLADAVLITTAHAWQHQGKTLFISRKTYRIDGSGQMAITVDVEVASDTPHPARIGLNCQLAQVAERVNWLGLGPQENYPDRLTAACFDRWDLPLSDMYTPYVFPSENGLRCGTRELNYGPHQWRGDFQFNISRYSQQQLMETSHRHLLHAEEGTWLNIDGFHMGIGGDDSWSPSVSAEFQLSAGRYHYQLVWCQK

SEQ ID NO: 30 - protein, 264 aa, Escherichia coli [sequence omitted]

SEQ ID NO: 31 - DNA, 70 bp, Escherichia coli
  source 1..70: mol_type = genomic DNA
tctgggcatatcgtcgcagcccacagcaacacgtttcctgaggaaccatgattccggggatccgtcgacc

SEQ ID NO: 32 - protein, 291 aa, Escherichia coli
MTSSYLHFPEFDPVIFSIGPVALHWYGLMYLVGFIFAMWLATRRANRPGSGWTKNEVENLLYAGFLGVFLGGRIGYVLFYNFPQFMADPLYLFRVWDGGMSFHGGLIGVIVVMIIFARRTKRSFFQVSDFIAPLIPFGLGAGRLGNFINGELWGRVDPNFPFAMLFPGSRTEDILLLQTNPQWQSIFDTYGVLPRHPSQLYELLLEGVVLFIILNLYIRKPRPMGAVSGLFLIGYGAFRIIVEFFRQPDAQFTGAWVQYISMGQILSIPMIVAGVIMMVWAYRRSPQQHVS

SEQ ID NO: 33 - DNA, 40 bp, Escherichia coli
  source 1..40: mol_type = genomic DNA
cagtcagtcaggcgcctcctcaacctgtatattcgtaaac

SEQ ID NO: 34 - DNA, 5877 bp, Escherichia coli; identical to SEQ ID NO: 1
  source 1..5877: mol_type = genomic DNA

SEQ ID NO: 35 - protein, 455 aa, Escherichia coli
MFGIIISVIVLITMGYLILKNYKPQVVLAAAGIFLMMCGVWLGFGGVLDPTKSSGYLIVDIYNEILRMLSNRIAGLGLSIMAVGGYARYMERIGASRAMVSLLSRPLKLIRSPYIILSATYVIGQIMAQFITSASGLGMLLMVTLFPTLVSLGVSRLSAVAVIATTMSIEWGILETNSIFAAQVAGMKIATYFFHYQLPVASCVIISVAISHFFVQRAFDKKDKNINHEQAEQKALDNVPPLYYAILPVMPLILMLGSLFLAHVGLMQSELHLVVVMLLSLTVTMFVEFFRKHNLRETMDDVQAFFDGMGTQFANVVTLVVAGEIFAKGLTTIGTVDAVIRGAEHSGLGGIGVMIIMALVIAICAIVMGSGNAPFMSFASLIPNIAAGLHVPAVVMIMPMHFATTLARAVSPITAVVVVTSGIAGVSPFAVVKRTAIPMAVGFVVNMIATITLFY

SEQ ID NO: 36 - protein, 263 aa, Escherichia coli
MGLMNAFDSQTEDSSPAIGRNLRSRPLARKKLSEMVEEELEQMIRRREFGEGEQLPSERELMAFFNVGRPSVREALAALKRKGLVQINNGERARVSRPSADTIIGELSGMAKDFLSHPGGIAHFEQLRLFFESSLVRYAAEHATDEQIDLLAKALEINSQSLDNNAAFIRSDVDFHRVLAEIPGNPIFMAIHVALLDWLIAARPTVTDQALHEHNNVSYQQHIAIVDAIRRHDPDEADRALQSHLNSVSATWHAFGQTTNKKK

SEQ ID NO: 37 - protein, 297 aa, Escherichia coli
MATNLRGVMAALLTPFDQQQALDKASLRRLVQFNIQQGIDGLYVGGSTGEAFVQSLSEREQVLEIVAEEAKGKIKLIAHVGCVSTAESQQLAASAKRYGFDAVSAVTPFYYPFSFEEHCDHYRAIIDSADGLPMVVYNIPALSGVKLTLDQINTLVTLPGVGALKQTSGDLYQMEQIRREHPDLVLYNGYDEIFASGLLAGADGGIGSTYNIMGWRYQGIVKALKEGDIQTAQKLQTECNKVIDLLIKTGVFRGLKTVLHYMDVVSVPLCRKPFGPVDEKYLPELKALAQQLMQERG

SEQ ID NO: 38 - protein, 496 aa, Escherichia coli
MSTTTQNIPWYRHLNRAQWRAFSAAWLGYLLDGFDFVLIALVLTEVQGEFGLTTVQAASLISAAFISRWFGGLMLGAMGDRYGRRLAMVTSIVLFSAGTLACGFAPGYITMFIARLVIGMGMAGEYGSSATYVIESWPKHLRNKASGFLISGFSVGAVVAAQVYSLVVPVWGWRALFFIGILPIIFALWLRKNIPEAEDWKEKHAGKAPVRTMVDILYRGEHRIANIVMTLAAATALWFCFAGNLQNAAIVAVLGLLCAAIFISFMVQSAGKRWPTGVMLMVVVLFAFLYSWPIQALLPTYLKTDLAYNPHTVANVLFFSGFGAAVGCCVGGFLGDWLGTRKAYVCSLLASQLLIIPVFAIGGANVWVLGLLLFFQQMLGQGIAGILPKLIGGYFDTDQRAAGLGFTYNVGALGGALAPIIGALIAQRLDLGTALASLSFSLTFVVILLIGLDMPSRVQRWLRPEALRTHDAIDGKPFSGAVPFGSAKNDLVKTKS

SEQ ID NO: 39 - protein, 229 aa, Escherichia coli
MSLLAQLDQKIAANGGLIVSCQPVPDSPLDKPEIVAAMALAAEQAGAVAIRIEGVANLQATRAVVSVPIIGIVKRDLEDSPVRITAYIEDVDALAQAGADIIAIDGTDRPRPVPVETLLARIHHHGLLAMTDCSTPEDGLACQKLGAEIIGTTLSGYTTPETPEEPDLALVKTLSDAGCRVIAEGRYNTPAQAADAMRHGAWAVTVGSAITRLEHICQWYNTAMKKAVL

SEQ ID NO: 40 - protein, 291 aa, Escherichia coli
MTTLAIDIGGTKLAAALIGADGQIRDRRELPTPASQTPEALRDALSALVSPLQAHAQRVAIASTGIIRDGSLLALNPHNLGGLLHFPLVKTLEQLTNLPTIAINDAQAAAWAEFQALDGDITDMVFITVSTGVGGGVVSGCKLLTGPGGLAGHIGHTLADPHGPVCGCGRTGCVEAIASGRGIAAAAQGELAGADAKTIFTRAGQGDEQAQQLIHRSARTLARLIADIKATTDCQCVVVGGSVGLAEGYLALVETYLAQEPAAFHVDLLAAHYRHDAGLLGAALLAQGEKL

SEQ ID NO: 41 - protein, 154 aa, Escherichia coli
MMMGEVQSLPSAGLHPALQDALTLALAARPQEKAPGRYELQGDNIFMNVMTFNTQSPVEKKAELHEQYIDIQLLLNGEERILFGMAGTARQCEEFHHEDDYQLCSTIDNEQAIILKPGMFAVFMPGEPHKPGCVVGEPGEIKKVVVKVKADLMA

SEQ ID NO: 42 - DNA, 5861 bp, Escherichia coli
  source 1..5861: mol_type = genomic DNA
gaacattgttgaactccgtgtcaaaagaaaacggtcaatcccataaacggcagattgaaaacaacgatgttatattttttgcaaggctatttatggtgcggatgtcgtgtttttaattgtaggtgaggtgatttttcattaaaaaatatgcgcttatgattattttgtaagaacacattcataatattcataatgctcgtgaatagtcttataaataattcaaacgggatgtttttatctgcgttacattaatttttcgcaatagttaattattccgttaattatggtaatgatgaggcacaaagagaaaaccctgccattttcccctactttcaatcctgtgataggatgtcactgatgatgttaatcacactgaccttacagaatgggccttatgaacgcatttgattcgcaaaccgaagattcttcacctgcaattggtcgcaacttgcgtagccgcccgctggcgcgtaaaaaactctccgaaatggtggaagaagagctggaacagatgatccgccgtcgtgaatttggcgaaggtgaacaattaccgtctgaacgcgaactgatggcgttctttaacgtcgggcgtccttcggtgcgtgaagcgctggcagcgttaaaacgcaaaggtctggtgcaaataaacaacggcgaacgcgctcgcgtctcgcgtccttctgcggacactatcatcggtgagctttccggcatggcgaaagatttcctttctcatcccggtgggattgcccatttcgaacaattacgtctgttctttgaatccagtctggtgcgctatgcggctgaacatgccaccgatgagcaaatcgatttgctggcaaaagcactggaaatcaacagtcagtcgctggataacaacgcggcattcattcgttcagacgttgatttccaccgcgtgctggcggagatccccggtaacccaatcttcatggcgatccacgttgccctgctcgactggcttattgccgcacgcccaacggttaccgatcaggcactgcacgaacataacaacgttagttatcaacagcatattgcgatcgttgatgcgatccgccgtcatgatcctgacgaagccgatcgtgcgttgcaatcgcatctcaacagcgtctctgctacctggcacgctttcggtcagaccaccaacaaaaagaaataatgccactttagtgaagcagatcgcattataagctttctgtatggggtgttgcttaattgatctggtataacaggtataaaggtatatcgtttatcagacaagcatcacttcagaggtatttatggcaacgaatttacgtggcgtaatggctgcactcctgactccttttgaccaacaacaagcactggataaagcgagtctgcgtcgcctggttcagttcaatattcagcagggcatcgacggtttatacgtgggtggttcgaccggcgaggcctttgtacaaagcctttccgagcgtgaacaggtactggaaatcgtcgccgaagaggcgaaaggtaagattaaactcatcgcccacgtcggttgcgtcagcaccgccgaaagccaacaacttgcggcatcggctaaacgttatggcttcgatgccgtctccgccgtcacgccgttctactatcctttcagctttgaagaacactgcgatcactatcgggcaattattgattcggcggatggtttgccgatggtggtgtacaacattccagccctgagtggggtaaaactgaccctggatcagatcaacacacttgttacattgcctggcgtaggtgcgctgaaacagacctctggcgatctctatcagatggagcagatccgtcgtgaacatcctgatcttgtgctctataacggttacgacgaaatcttcgcctctggtctgctggcgggcgctgatggtggtatcggcagtacctacaacatcatgggctggcgctatcaggggatcgttaaggcgctgaaagaaggcgatatccagaccgcgcagaaactgcaaactgaatgcaataaagtcattgatttactgatcaaaacgggcgtattccgcggcctgaaaactgtcctccattatatggatgtcgtttctgtgccgctgtgccgcaaaccgtttggaccggtagatgaaaaatatctgccagaactgaaggcgctggcccagcagttgatgcaagagcgcgggtgagttgtttcccctcgctcgcccctaccgggtgaggggaaataaacgcatctgtaccctacaattttcataccaaagcgtgtgggcatcgcccaccgcgggagactcacaatgagtactacaacccagaatatcccgtggtatcgccatctcaaccgtgcacaatggcgcgcattttccgctgcctggttgggatatctgcttgacggttttgatttcgttttaatcgccctggtactcaccgaagtacaaggtgaattcgggctgacgacggtgcaggcggcaagtctgatctctgcagcctttatctctcgctggttcggcggcctgatgctcggcgctatgggtgaccgctacgggcgtcgtctggcaatggtcaccagcatcgttctcttctcggccgggacgctggcctgcggctttgcgccaggctacatcaccatgtttatcgctcgtctggtcatcggcatggggatggcgggtgaatacggttccagcgccacctatgtcattgaaagctggccaaaacatctgcgtaacaaagccagtggttttttgatttcaggcttctctgtgggggccgtcgttgccgctcaggtctatagcctggtggttccggtctggggctggcgtgcgctgttctttatcggcattttgccaatcatctttgctctctggctgcgtaaaaacatcccggaagcggaagactggaaagagaaacacgcaggtaaagcaccagtacgcacaatggtggatattctctaccgtggtgaacatcgcattgccaatatcgtaatgacactggcggcggctactgcgctgtggttctgcttcgccggtaacctgcaaaatgccgcgatcgtcgctgttcttgggctgttatgcgccgcaatctttatcagctttatggtgcagagtgcaggcaaacgctggccaacgggcgtaatgctgatggtggtcgtgttgtttgctttcctctactcatggccgattcaggcgctgctgccaacgtatctgaaaaccgatctggcttataacccgcatactgtagccaatgtgctgttctttagtggctttggcgcggcggtgggatgctgcgtaggtggcttcctcggtgactggctgggaacccgcaaagcgtacgtttgtagcctgctggcctcgcagctgctgattattccggtatttgcgattggcggcgcaaacgtctgggtgctcggtctgttactgttcttccagcaaatgcttggacaagggatcgccgggatcttaccaaaactgattggcggttatttcgataccgaccagcgtgcagcgggcctgggctttacctacaacgttggcgcattgggcggtgcactggccccaatcatcggcgcgttgatcgctcaacgtctggatctgggtactgcgctggcatcgctctcgttcagtctgacgttcgtggtgatcctgctgattgggctggatatgccttctcgcgttcagcgttggttgcgcccggaagcgttgcgtactcatgacgctatcgacggtaaaccattcagcggtgccgtgccgtttggcagcgccaaaaacgatttagtcaaaaccaaaagttaatcctgttgcccggtctatgtaccgggcctttcgctaagggaagatgtatgtcgttacttgcacaactggatcaaaaaatcgctgctaacggtggcctgattgtctcctgccagccggttccggacagcccgctcgataaacccgaaatcgtcgccgccatggcattagcggcagaacaggcgggcgcggttgccattcgcattgaaggtgtggcaaatctgcaagccacgcgtgcggtggtgagcgtgccgattattggaattgtgaaacgcgatctggaggattctccggtacgcatcacggcctatattgaagatgttgatgcgctggcgcaggcgggcgcggacattatcgccattgacggcaccgaccgcccgcgtccggtgcctgttgaaacgctgctggcacgtattcaccatcacggtttactggcgatgaccgactgctcaacgccggaagacggcctggcatgccaaaagctgggagccgaaattattggcactacgctttctggctataccacgcctgaaacgccagaagagccggatctggcgctggtgaaaacgttgagcgacgccggatgtcgggtgattgccgaagggcgttacaacacgcctgctcaggcggcggatgcgatgcgccacggcgcgtgggcggtgacggtcggttctgcaatcacgcgtcttgagcacatttgtcagtggtacaacacagcgatgaaaaaggcggtgctatgaccacactggcgattgatatcggcggtactaaacttgccgccgcgctgattggcgctgacgggcagatccgcgatcgtcgtgaacttcctacgccagccagccagacaccagaagccttgcgtgatgccttatccgcattagtctctccgttgcaagctcatgcgcagcgggttgccatcgcttcgaccgggataatccgtgacggcagcttgctggcgcttaatccgcataatcttggtggattgctacactttccgttagtcaaaacgctggaacaacttaccaatttgccgaccattgccattaacgacgcgcaggccgcagcatgggcggagtttcaggcgctggatggcgatataaccgatatggtctttatcaccgtttccaccggcgttggcggcggtgtagtgagcggctgcaaactgcttaccggccctggcggtctggcggggcatatcgggcatacgcttgccgatccacacggcccagtctgcggctgtggacgcacaggttgcgtggaagcgattgcttctggtcgcggcattgcagcggcagcgcagggggagttggctggcgcggatgcgaaaactattttcacgcgcgccgggcagggtgacgagcaggcgcagcagctgattcaccgctccgcacgtacgcttgcaaggctgatcgctgatattaaagccacaactgattgccagtgcgtggtggtcggtggcagcgttggtctggcagaagggtatctggcgctggtggaaacgtatctggcgcaggagccagcggcatttcatgttgatttactggcggcgcattaccgccatgatgcaggtttacttggggctgcgctgttggcccagggagaaaaattatgatgatgggtgaagtacagtcattaccgtctgctgggttacatcctgcgttacaggacgcgttaacgctggcattagctgccagaccgcaagaaaaagcgccgggtcgttacgaattacagggcgacaatatctttatgaatgtcatgacgtttaacactcaatcgcccgtcgagaaaaaagcggaattgcacgagcaatacattgatatccagctgttattaaacggtgaggaacggattctgtttggcatggcaggcactgcgcgtcagtgtgaagagttccaccatgaggatgattatcagctttgcagcaccattgataacgagcaagccatcatcttaaaaccgggaatgttcgccgtgtttatgccaggtgaaccgcataaaccaggatgcgttgtcggcgagcctggagagattaaaaaggttgtggtgaaggttaaggctgatttaatggcttaa

SEQ ID NO: 43 - protein, 264 aa, Escherichia coli
MKQYLELMQKVLDEGTQKNDRTGTGTLSIFGHQMRFNLQDGFPLVTTKRCHLRSIIHELLWFLQGDTNIAYLHENNVTIWDEWADENGDLGPVYGKQWRAWPTPDGRHIDQITTVLNQLKNDPDSRRIIVSAWNVGELDKMALAPCHAFFQFYVADGKLSCQLYQRSCDVFLGLPFNIASYALLVHMMAQQCDLEVGDFVWTGGDTHLYSNHMDQTHLQLSREPRPLPKLIIKRKPESIFDYRFEDFEIEGYDPHPGIKAPVAI